European Patent Application EP 4 512 831 A1, published February 26, 2025. Title: ANTIBODY COMPRISING IGG FC REGION VARIANT, AND USE THEREOF. Applicant: Nanjing RegeneCore Biotech Co., Ltd. The sequence listing filed with the application follows.

SEQUENCE LISTING (152 sequences)

SEQ ID NO: 1 - protein, 232 aa, synthetic construct
EPKSCDKTHTCPPCPAPELLGGPSVFLFPPKPKDTLMISRTPEVTCVVVDVSHEDPEVKFNWYVDGVEVHNAKTKPREEQYNSTYRVVSVLTVLHQDWLNGKEYKCKVSNKALPAPIEKTISKAKGQPREPQVYTLPPSRDELTKNQVSLWCLVKGFYPSDIAVEWESNGQPENNYKTTPPVLVSDGSFTLYSKLTVDKSRWQQGNVFSCSVMHEALHNHYTQKSLSLSPGK

SEQ ID NO: 2 - protein, 232 aa, synthetic construct
EPKSCDKTHTCPPCPAPELLGGPSVFLFPPKPKDTLMISRTPEVTCVVVDVSHEDPEVKFNWYVDGVEVHNAKTKPREEQYNSTYRVVSVLTVLHQDWLNGKEYKCKVSNKALPAPIEKTISKAKGQPREPQVYTLPPSRDKLTKNQVSLWCLVKGFYPSDIAVEWESNGQPENNYKTTPPVLKSDGSFFLYSKLTVDKSRWQQGNVFSCSVMHEALHNHYTQKSLSLSPGK

SEQ ID NO: 3 - protein, 232 aa, synthetic construct
EPKSCDKTHTCPPCPAPELLGGPSVFLFPPKPKDTLMISRTPEVTCVVVDVSHEDPEVKFNWYVDGVEVHNAKTKPREEQYNSTYRVVSVLTVLHQDWLNGKEYKCKVSNKALPAPIEKTISKAKGQPREPQVYTLPPSRDELTKNQVSLVCLVKGFYPSDIAVEWESNGQPENNYKTTPPVLVSDGSFTLYSKLTVDKSRWQQGNVFSCSVMHEALHNHYTQKSLSLSPGK

SEQ ID NO: 4 - protein, 232 aa, synthetic construct
EPKSCDKTHTCPPCPAPELLGGPSVFLFPPKPKDTLMISRTPEVTCVVVDVSHEDPEVKFNWYVDGVEVHNAKTKPREEQYNSTYRVVSVLTVLHQDWLNGKEYKCKVSNKALPAPIEKTISKAKGQPREPQVYTLPPSRDKLTKNQVSLVCLVKGFYPSDIAVEWESNGQPENNYKTTPPVLKSDGSFFLYSKLTVDKSRWQQGNVFSCSVMHEALHNHYTQKSLSLSPGK

SEQ ID NO: 5 - protein, 232 aa, synthetic construct
EPKSCDKTHTCPPCPAPELLGGPSVFLFPPKPKDTLMISRTPEVTCVVVDVSHEDPEVKFNWYVDGVEVHNAKTKPREEQYNSTYRVVSVLTVLHQDWLNGKEYKCKVSNKALPAPIEKTISKAKGQPREPQVYTLPPSRKELTKNQVSLWCLVKGFYPSDIAVEWESNGQPENNYKTTPPVLDSDGSFFLYSKLTVDKSRWQQGNVFSCSVMHEALHNHYTQKSLSLSPGK

SEQ ID NO: 6 - protein, 232 aa, synthetic construct
EPKSCDKTHTCPPCPAPELLGGPSVFLFPPKPKDTLMISRTPEVTCVVVDVSHEDPEVKFNWYVDGVEVHNAKTKPREEQYNSTYRVVSVLTVLHQDWLNGKEYKCKVSNKALPAPIEKTISKAKGQPREPQVYTLPPSRDDLTKNQVSLWCLVKGFYPSDIAVEWESNGQPENNYKTTPPVLDSDGSFFLYSKLTVDKSRWQQGNVFSCSVMHEALHNHYTQKSLSLSPGK

SEQ ID NO: 7 - protein, 232 aa, synthetic construct
EPKSCDKTHTCPPCPAPELLGGPSVFLFPPKPKDTLMISRTPEVTCVVVDVSHEDPEVKFNWYVDGVEVHNAKTKPREEQYNSTYRVVSVLTVLHQDWLNGKEYKCKVSNKALPAPIEKTISKAKGQPREPRVYTLPPSRDELTKNQVSLWCLVKGFYPSDIAVEWESNGQPENNYKTTPPVLDSDGSFFLYSKLTVDKSRWQQGNVFSCSVMHEALHNHYTQKSLSLSPGK

SEQ ID NO: 8 - protein, 232 aa, synthetic construct
EPKSCDKTHTCPPCPAPELLGGPSVFLFPPKPKDTLMISRTPEVTCVVVDVSHEDPEVKFNWYVDGVEVHNAKTKPREEQYNSTYRVVSVLTVLHQDWLNGKEYKCKVSNKALPAPIEKTISKAKGQPREPQVYTLPPSRKELTKNQVSLVCLVKGFYPSDIAVEWESNGQPENNYKTTPPVLDSDGSFFLYSKLTVDKSRWQQGNVFSCSVMHEALHNHYTQKSLSLSPGK

SEQ ID NO: 9 - protein, 232 aa, synthetic construct
EPKSCDKTHTCPPCPAPELLGGPSVFLFPPKPKDTLMISRTPEVTCVVVDVSHEDPEVKFNWYVDGVEVHNAKTKPREEQYNSTYRVVSVLTVLHQDWLNGKEYKCKVSNKALPAPIEKTISKAKGQPREPQVYTLPPSRDDLTKNQVSLVCLVKGFYPSDIAVEWESNGQPENNYKTTPPVLDSDGSFFLYSKLTVDKSRWQQGNVFSCSVMHEALHNHYTQKSLSLSPGK

SEQ ID NO: 10 - protein, 232 aa, synthetic construct
EPKSCDKTHTCPPCPAPELLGGPSVFLFPPKPKDTLMISRTPEVTCVVVDVSHEDPEVKFNWYVDGVEVHNAKTKPREEQYNSTYRVVSVLTVLHQDWLNGKEYKCKVSNKALPAPIEKTISKAKGQPREPRVYTLPPSRDELTKNQVSLVCLVKGFYPSDIAVEWESNGQPENNYKTTPPVLDSDGSFFLYSKLTVDKSRWQQGNVFSCSVMHEALHNHYTQKSLSLSPGK

SEQ ID NO: 11 - protein, 232 aa, synthetic construct
EPKSCDKTHTCPPCPAPELLGGPSVFLFPPKPKDTLMISRTPEVTCVVVDVSHEDPEVKFNWYVDGVEVHNAKTKPREEQYNSTYRVVSVLTVLHQDWLNGKEYKCKVSNKALPAPIEKTISKAKGQPREPQVYTLPPSRDELTKNQVSLWCLVKGFYPSDIAVEWESNGQPENNYKTTPPVLDSDGSFFLYSWLTVDKSRWQQGNVFSCSVMHEALHNHYTQKSLSLSPGK

SEQ ID NO: 12 - protein, 232 aa, synthetic construct
EPKSCDKTHTCPPCPAPELLGGPSVFLFPPKPKDTLMISRTPEVTCVVVDVSHEDPEVKFNWYVDGVEVHNAKTKPREEQYNSTYRVVSVLTVLHQDWLNGKEYKCKVSNKALPAPIEKTISKAKGQPREPQVYTLPPSRDELTKNQVSLWCLVEGFYPSDIAVEWESNGQPENNYKTTPPVLDSDGSFFLYSDLTVDKSRWQQGNVFSCSVMHEALHNHYTQKSLSLSPGK

SEQ ID NO: 13 - protein, 232 aa, synthetic construct
EPKSCDKTHTCPPCPAPELLGGPSVFLFPPKPKDTLMISRTPEVTCVVVDVSHEDPEVKFNWYVDGVEVHNAKTKPREEQYNSTYRVVSVLTVLHQDWLNGKEYKCKVSNKALPAPIEKTISKAKGQPREPQVYTLPPSRDELTKNQVSLVCLVKGFYPSDIAVEWESNGQPENNYKTTPPVLDSDGSFFLYSWLTVDKSRWQQGNVFSCSVMHEALHNHYTQKSLSLSPGK

SEQ ID NO: 14 - protein, 232 aa, synthetic construct
EPKSCDKTHTCPPCPAPELLGGPSVFLFPPKPKDTLMISRTPEVTCVVVDVSHEDPEVKFNWYVDGVEVHNAKTKPREEQYNSTYRVVSVLTVLHQDWLNGKEYKCKVSNKALPAPIEKTISKAKGQPREPQVYTLPPSRDELTKNQVSLVCLVEGFYPSDIAVEWESNGQPENNYKTTPPVLDSDGSFFLYSDLTVDKSRWQQGNVFSCSVMHEALHNHYTQKSLSLSPGK

SEQ ID NO: 15 - protein, 232 aa, synthetic construct
EPKSCDKTHTCPPCPAPELLGGPSVFLFPPKPKDTLMISRTPEVTCVVVDVSHEDPEVKFNWYVDGVEVHNAKTKPREEQYNSTYRVVSVLTVLHQDWLNGKEYKCKVSNKALPAPIEKTISKAKGQPREPQVYTLPPSRDELTKNQVSLWCLVKGFYPSDIAVEWESNGQPENNYKTTPPVLDSDGSFFLYSKLTVDKSRWQQGNVFSCSVMHEALHNHYTQESLSLSPGK

SEQ ID NO: 16 - protein, 232 aa, synthetic construct
EPKSCDKTHTCPPCPAPELLGGPSVFLFPPKPKDTLMISRTPEVTCVVVDVSHEDPEVKFNWYVDGVEVHNAKTKPREEQYNSTYRVVSVLTVLHQDWLNGKEYKCKVSNKALPAPIEKTISKAKGQPREPQVYTLPPSRDELTKNQVSLWCLVYGFYPSDIAVEWESNGQPENNYKTTPPVLDSDGSFFLYSKLTVDKSRWQQGNVFSCSVMHEALHNHYTQKSLSLSPGK

SEQ ID NO: 17 - protein, 232 aa, synthetic construct
EPKSCDKTHTCPPCPAPELLGGPSVFLFPPKPKDTLMISRTPEVTCVVVDVSHEDPEVKFNWYVDGVEVHNAKTKPREEQYNSTYRVVSVLTVLHQDWLNGKEYKCKVSNKALPAPIEKTISKAKGQPREPQVYTLPPSRDELTDNQVSLWCLVKGFYPSDIAVEWESNGQPENNYKTTPPVLDSDGSFFLYSKLTVDKSRWQQGNVFSCSVMHEALHNHYTQKSLSLSPGK

SEQ ID NO: 18 - protein, 232 aa, synthetic construct
EPKSCDKTHTCPPCPAPELLGGPSVFLFPPKPKDTLMISRTPEVTCVVVDVSHEDPEVKFNWYVDGVEVHNAKTKPREEQYNSTYRVVSVLTVLHQDWLNGKEYKCKVSNKALPAPIEKTISKAKGQPREPQVYTLPPSRDELTKNQVSLVCLVKGFYPSDIAVEWESNGQPENNYKTTPPVLDSDGSFFLYSKLTVDKSRWQQGNVFSCSVMHEALHNHYTQESLSLSPGK

SEQ ID NO: 19 - protein, 232 aa, synthetic construct
EPKSCDKTHTCPPCPAPELLGGPSVFLFPPKPKDTLMISRTPEVTCVVVDVSHEDPEVKFNWYVDGVEVHNAKTKPREEQYNSTYRVVSVLTVLHQDWLNGKEYKCKVSNKALPAPIEKTISKAKGQPREPQVYTLPPSRDELTKNQVSLTCLVYGFYPSDIAVEWESNGQPENNYKTTPPVLDSDGSFFLASKLTVDKSRWQQGNVFSCSVMHEALHNHYTQKSLSLSPGK

SEQ ID NO: 20 - protein, 232 aa, synthetic construct
EPKSCDKTHTCPPCPAPELLGGPSVFLFPPKPKDTLMISRTPEVTCVVVDVSHEDPEVKFNWYVDGVEVHNAKTKPREEQYNSTYRVVSVLTVLHQDWLNGKEYKCKVSNKALPAPIEKTISKAKGQPREPQVYTLPPSRDELTDNQVSLVCLVKGFYPSDIAVEWESNGQPENNYKTTPPVLDSDGSFFLYSKLTVDKSRWQQGNVFSCSVMHEALHNHYTQKSLSLSPGK

SEQ ID NO: 21 - protein, 232 aa, synthetic construct
EPKSCDKTHTCPPCPAPELLGGPSVFLFPPKPKDTLMISRTPEVTCVVVDVSHEDPEVKFNWYVDGVEVHNAKTKPREEQYNSTYRVVSVLTVLHQDWLNGKEYKCKVSNKALPAPIEKTISKAKGQPREPQVYTLPPSRKELTKNQVSLTCLVKGFYPSDIAVEWESNGQPENNYKTTPPVLVSDGSFTLYSKLTVDKSRWQQGNVFSCSVMHEALHNHYTQKSLSLSPGK

SEQ ID NO: 22 - protein, 232 aa, synthetic construct
EPKSCDKTHTCPPCPAPELLGGPSVFLFPPKPKDTLMISRTPEVTCVVVDVSHEDPEVKFNWYVDGVEVHNAKTKPREEQYNSTYRVVSVLTVLHQDWLNGKEYKCKVSNKALPAPIEKTISKAKGQPREPQVYTLPPSRDKLTKNQVSLTCLVKGFYPSDIAVEWESNGQPENNYKTTPPVLVSDGSFTLYSKLTVDKSRWQQGNVFSCSVMHEALHNHYTQKSLSLSPGK

SEQ ID NO: 23 - protein, 232 aa, synthetic construct
EPKSCDKTHTCPPCPAPELLGGPSVFLFPPKPKDTLMISRTPEVTCVVVDVSHEDPEVKFNWYVDGVEVHNAKTKPREEQYNSTYRVVSVLTVLHQDWLNGKEYKCKVSNKALPAPIEKTISKAKGQPREPQVYTLPPSRDDLTKNQVSLTCLVKGFYPSDIAVEWESNGQPENNYKTTPPVLVSDGSFTLYSKLTVDKSRWQQGNVFSCSVMHEALHNHYTQKSLSLSPGK

SEQ ID NO: 24 - protein, 232 aa, synthetic construct
EPKSCDKTHTCPPCPAPELLGGPSVFLFPPKPKDTLMISRTPEVTCVVVDVSHEDPEVKFNWYVDGVEVHNAKTKPREEQYNSTYRVVSVLTVLHQDWLNGKEYKCKVSNKALPAPIEKTISKAKGQPREPQVYTLPPSRKDLTKNQVSLTCLVKGFYPSDIAVEWESNGQPENNYKTTPPVLDSDGSFFLASKLTVDKSRWQQGNVFSCSVMHEALHNHYTQKSLSLSPGK

SEQ ID NO: 25 - protein, 232 aa, synthetic construct
EPKSCDKTHTCPPCPAPELLGGPSVFLFPPKPKDTLMISRTPEVTCVVVDVSHEDPEVKFNWYVDGVEVHNAKTKPREEQYNSTYRVVSVLTVLHQDWLNGKEYKCKVSNKALPAPIEKTISKAKGQPREPQVYTLPPSRDDLTKNQVSLTCLVKGFYPSDIAVEWESNGQPENNYKTTPPVLKSDGSFFLYSKLTVDKSRWQQGNVFSCSVMHEALHNHYTQKSLSLSPGK

SEQ ID NO: 26 - protein, 232 aa, synthetic construct
EPKSCDKTHTCPPCPAPELLGGPSVFLFPPKPKDTLMISRTPEVTCVVVDVSHEDPEVKFNWYVDGVEVHNAKTKPREEQYNSTYRVVSVLTVLHQDWLNGKEYKCKVSNKALPAPIEKTISKAKGQPREPQVYTLPPSRKKLTKNQVSLTCLVKGFYPSDIAVEWESNGQPENNYKTTPPVLVSDGSFTLYSKLTVDKSRWQQGNVFSCSVMHEALHNHYTQKSLSLSPGK

SEQ ID NO: 27 - protein, 232 aa, synthetic construct
EPKSCDKTHTCPPCPAPELLGGPSVFLFPPKPKDTLMISRTPEVTCVVVDVSHEDPEVKFNWYVDGVEVHNAKTKPREEQYNSTYRVVSVLTVLHQDWLNGKEYKCKVSNKALPAPIEKTISKAKGQPREPQVYTLPPSRKDLTKNQVSLTCLVKGFYPSDIAVEWESNGQPENNYKTTPPVLVSDGSFTLYSKLTVDKSRWQQGNVFSCSVMHEALHNHYTQKSLSLSPGK

SEQ ID NO: 28 - protein, 232 aa, synthetic construct
EPKSCDKTHTCPPCPAPELLGGPSVFLFPPKPKDTLMISRTPEVTCVVVDVSHEDPEVKFNWYVDGVEVHNAKTKPREEQYNSTYRVVSVLTVLHQDWLNGKEYKCKVSNKALPAPIEKTISKAKGQPREPQVYTLPPSRKDLTKNQVSLTCLVKGFYPSDIAVEWESNGQPENNYKTTPPVLKSDGSFFLYSKLTVDKSRWQQGNVFSCSVMHEALHNHYTQKSLSLSPGK

SEQ ID NO: 29 - protein, 232 aa, synthetic construct
EPKSCDKTHTCPPCPAPELLGGPSVFLFPPKPKDTLMISRTPEVTCVVVDVSHEDPEVKFNWYVDGVEVHNAKTKPREEQYNSTYRVVSVLTVLHQDWLNGKEYKCKVSNKALPAPIEKTISKAKGQPREPRVYTLPPSRKELTKNQVSLTCLVKGFYPSDIAVEWESNGQPENNYKTTPPVLDSDGSFFLASKLTVDKSRWQQGNVFSCSVMHEALHNHYTQKSLSLSPGK

SEQ ID NO: 30 - protein, 232 aa, synthetic construct
EPKSCDKTHTCPPCPAPELLGGPSVFLFPPKPKDTLMISRTPEVTCVVVDVSHEDPEVKFNWYVDGVEVHNAKTKPREEQYNSTYRVVSVLTVLHQDWLNGKEYKCKVSNKALPAPIEKTISKAKGQPREPRVYTLPPSRDKLTKNQVSLTCLVKGFYPSDIAVEWESNGQPENNYKTTPPVLDSDGSFFLASKLTVDKSRWQQGNVFSCSVMHEALHNHYTQKSLSLSPGK

SEQ ID NO: 31 - protein, 232 aa, synthetic construct
EPKSCDKTHTCPPCPAPELLGGPSVFLFPPKPKDTLMISRTPEVTCVVVDVSHEDPEVKFNWYVDGVEVHNAKTKPREEQYNSTYRVVSVLTVLHQDWLNGKEYKCKVSNKALPAPIEKTISKAKGQPREPRVYTLPPSRDELTKNQVSLTCLVKGFYPSDIAVEWESNGQPENNYKTTPPVLKSDGSFFLYSKLTVDKSRWQQGNVFSCSVMHEALHNHYTQKSLSLSPGK

SEQ ID NO: 32 - protein, 232 aa, synthetic construct
EPKSCDKTHTCPPCPAPELLGGPSVFLFPPKPKDTLMISRTPEVTCVVVDVSHEDPEVKFNWYVDGVEVHNAKTKPREEQYNSTYRVVSVLTVLHQDWLNGKEYKCKVSNKALPAPIEKTISKAKGQPREPRVYTLPPSRDDLTKNQVSLTCLVKGFYPSDIAVEWESNGQPENNYKTTPPVLDSDGSFFLASKLTVDKSRWQQGNVFSCSVMHEALHNHYTQKSLSLSPGK

SEQ ID NO: 33 - protein, 232 aa, synthetic construct
EPKSCDKTHTCPPCPAPELLGGPSVFLFPPKPKDTLMISRTPEVTCVVVDVSHEDPEVKFNWYVDGVEVHNAKTKPREEQYNSTYRVVSVLTVLHQDWLNGKEYKCKVSNKALPAPIEKTISKAKGQPREPQVYTLPPSRDELTKNQVSLDCLVKGFYPSDIAVEWESNGQPENNYKTTPPVLDSDGSFFLYSKLTVDKSRWQQGNVFSCSVMHEALHNHYTQKSLSLSPGK

SEQ ID NO: 34 - protein, 232 aa, synthetic construct
EPKSCDKTHTCPPCPAPELLGGPSVFLFPPKPKDTLMISRTPEVTCVVVDVSHEDPEVKFNWYVDGVEVHNAKTKPREEQYNSTYRVVSVLTVLHQDWLNGKEYKCKVSNKALPAPIEKTISKAKGQPREPQVYTLPPSRVELTKNQVSLTCLVKGFYPSDIAVEWESNGQPENNYKTTPPVLDSDGSFFLYSKLTVDKSRWQQGNVFSCSVMHEALHNHYTQKSLSLSPGK

SEQ ID NO: 35 - protein, 232 aa, synthetic construct
EPKSCDKTHTCPPCPAPELLGGPSVFLFPPKPKDTLMISRTPEVTCVVVDVSHEDPEVKFNWYVDGVEVHNAKTKPREEQYNSTYRVVSVLTVLHQDWLNGKEYKCKVSNKALPAPIEKTISKAKGQPREPQVYTLPPSRDVLTKNQVSLTCLVKGFYPSDIAVEWESNGQPENNYKTTPPVLDSDGSFFLYSKLTVDKSRWQQGNVFSCSVMHEALHNHYTQKSLSLSPGK

SEQ ID NO: 36 - protein, 232 aa, synthetic construct
EPKSCDKTHTCPPCPAPELLGGPSVFLFPPKPKDTLMISRTPEVTCVVVDVSHEDPEVKFNWYVDGVEVHNAKTKPREEQYNSTYRVVSVLTVLHQDWLNGKEYKCKVSNKALPAPIEKTISKAKGQPREPQVYTLPPSRDELTKNQVSLTCLVKGFYPSDIAVEWESNGQPENNYKTWPPVLDSDGSFFLYSKLTVDKSRWQQGNVFSCSVMHEALHNHYTQKSLSLSPGK

SEQ ID NO: 37 - protein, 232 aa, synthetic construct
EPKSCDKTHTCPPCPAPELLGGPSVFLFPPKPKDTLMISRTPEVTCVVVDVSHEDPEVKFNWYVDGVEVHNAKTKPREEQYNSTYRVVSVLTVLHQDWLNGKEYKCKVSNKALPAPIEKTISKAKGQPREPMVYTLPPSRDELTKNQVSLTCLVKGFYPSDIAVEWESNGQPENNYKTTPPVLDSDGSFFLYSKLTVDKSRWQQGNVFSCSVMHEALHNHYTQKSLSLSPGK

SEQ ID NO: 38 - protein, 232 aa, synthetic construct
EPKSCDKTHTCPPCPAPELLGGPSVFLFPPKPKDTLMISRTPEVTCVVVDVSHEDPEVKFNWYVDGVEVHNAKTKPREEQYNSTYRVVSVLTVLHQDWLNGKEYKCKVSNKALPAPIEKTISKAKGQPREPQVYTLPPSRDELTKNQVSLSCAVKGFYPSDIAVEWESNGQPENNYKTTPPVLDSDGSFFLVSWLTVDKSRWQQGNVFSCSVMHEALHNHYTQKSLSLSPGK

SEQ ID NO: 39 - protein, 232 aa, synthetic construct
EPKSCDKTHTCPPCPAPELLGGPSVFLFPPKPKDTLMISRTPEVTCVVVDVSHEDPEVKFNWYVDGVEVHNAKTKPREEQYNSTYRVVSVLTVLHQDWLNGKEYKCKVSNKALPAPIEKTISKAKGQPREPQVYTLPPSRDELTKNQVSLSCAVEGFYPSDIAVEWESNGQPENNYKTTPPVLDSDGSFFLVSDLTVDKSRWQQGNVFSCSVMHEALHNHYTQKSLSLSPGK

SEQ ID NO: 40 - protein, 232 aa, synthetic construct
EPKSCDKTHTCPPCPAPELLGGPSVFLFPPKPKDTLMISRTPEVTCVVVDVSHEDPEVKFNWYVDGVEVHNAKTKPREEQYNSTYRVVSVLTVLHQDWLNGKEYKCKVSNKALPAPIEKTISKAKGQPREPQVYTLPPSRDELTKNQVSLTCLVKGFYPSDIAVEWESNGQPENNYKTTPPVLDSDGSFFLASWLTVDKSRWQQGNVFSCSVMHEALHNHYTQKSLSLSPGK

SEQ ID NO: 41 - protein, 232 aa, synthetic construct
EPKSCDKTHTCPPCPAPELLGGPSVFLFPPKPKDTLMISRTPEVTCVVVDVSHEDPEVKFNWYVDGVEVHNAKTKPREEQYNSTYRVVSVLTVLHQDWLNGKEYKCKVSNKALPAPIEKTISKAKGQPREPQVYTLPPSRDELTKNQVSLTCLVEGFYPSDIAVEWESNGQPENNYKTTPPVLDSDGSFFLASDLTVDKSRWQQGNVFSCSVMHEALHNHYTQKSLSLSPGK

SEQ ID NO: 42 - protein, 232 aa, synthetic construct
EPKSCDKTHTCPPCPAPELLGGPSVFLFPPKPKDTLMISRTPEVTCVVVDVSHEDPEVKFNWYVDGVEVHNAKTKPREEQYNSTYRVVSVLTVLHQDWLNGKEYKCKVSNKALPAPIEKTISKAKGQPREPQVYTLPPSRDELTKNQVSLSCAVKGFYPSDIAVEWESNGQPENNYKTTPPVLDSDGSFFLVSKLTVDKSRWQQGNVFSCSVMHEALHNHYTQESLSLSPGK

SEQ ID NO: 43 - protein, 232 aa, synthetic construct
EPKSCDKTHTCPPCPAPELLGGPSVFLFPPKPKDTLMISRTPEVTCVVVDVSHEDPEVKFNWYVDGVEVHNAKTKPREEQYNSTYRVVSVLTVLHQDWLNGKEYKCKVSNKALPAPIEKTISKAKGQPREPQVYTLPPSRDELTKNQVSLSCAVYGFYPSDIAVEWESNGQPENNYKTTPPVLDSDGSFFLVSKLTVDKSRWQQGNVFSCSVMHEALHNHYTQKSLSLSPGK

SEQ ID NO: 44 - protein, 232 aa, synthetic construct
EPKSCDKTHTCPPCPAPELLGGPSVFLFPPKPKDTLMISRTPEVTCVVVDVSHEDPEVKFNWYVDGVEVHNAKTKPREEQYNSTYRVVSVLTVLHQDWLNGKEYKCKVSNKALPAPIEKTISKAKGQPREPQVYTLPPSRDELTDNQVSLSCAVKGFYPSDIAVEWESNGQPENNYKTTPPVLDSDGSFFLVSKLTVDKSRWQQGNVFSCSVMHEALHNHYTQKSLSLSPGK

SEQ ID NO: 45 - protein, 232 aa, synthetic construct
EPKSCDKTHTCPPCPAPELLGGPSVFLFPPKPKDTLMISRTPEVTCVVVDVSHEDPEVKFNWYVDGVEVHNAKTKPREEQYNSTYRVVSVLTVLHQDWLNGKEYKCKVSNKALPAPIEKTISKAKGQPREPQVYTLPPSRDELTKNQVSLTCLVKGFYPSDIAVEWESNGQPENNYKTTPPVLDSDGSFFLASKLTVDKSRWQQGNVFSCSVMHEALHNHYTQESLSLSPGK

SEQ ID NO: 46 - protein, 232 aa, synthetic construct; identical to SEQ ID NO: 19

SEQ ID NO: 47 - protein, 232 aa, synthetic construct
EPKSCDKTHTCPPCPAPELLGGPSVFLFPPKPKDTLMISRTPEVTCVVVDVSHEDPEVKFNWYVDGVEVHNAKTKPREEQYNSTYRVVSVLTVLHQDWLNGKEYKCKVSNKALPAPIEKTISKAKGQPREPQVYTLPPSRDELTDNQVSLTCLVKGFYPSDIAVEWESNGQPENNYKTTPPVLDSDGSFFLASKLTVDKSRWQQGNVFSCSVMHEALHNHYTQKSLSLSPGK

SEQ ID NO: 48 - protein, 232 aa, synthetic construct
EPKSCDKTHTCPPCPAPELLGGPSVFLFPPKPKDTLMISRTPEVTCVVVDVSHEDPEVKFNWYVDGVEVHNAKTKPREEQYNSTYRVVSVLTVLHQDWLNGKEYKCKVSNKALPAPIEKTISKAKGQPREPQVYTLPPSRDELTKNQVSLSCAVKGFYPSDIAVEWESNGQPENNYKTTPPVLVSDGSFTLVSKLTVDKSRWQQGNVFSCSVMHEALHNHYTQKSLSLSPGK

SEQ ID NO: 49 - protein, 232 aa, synthetic construct
EPKSCDKTHTCPPCPAPELLGGPSVFLFPPKPKDTLMISRTPEVTCVVVDVSHEDPEVKFNWYVDGVEVHNAKTKPREEQYNSTYRVVSVLTVLHQDWLNGKEYKCKVSNKALPAPIEKTISKAKGQPREPQVYTLPPSRDKLTKNQVSLSCAVKGFYPSDIAVEWESNGQPENNYKTTPPVLKSDGSFFLVSKLTVDKSRWQQGNVFSCSVMHEALHNHYTQKSLSLSPGK

SEQ ID NO: 50 - protein, 232 aa, synthetic construct
EPKSCDKTHTCPPCPAPELLGGPSVFLFPPKPKDTLMISRTPEVTCVVVDVSHEDPEVKFNWYVDGVEVHNAKTKPREEQYNSTYRVVSVLTVLHQDWLNGKEYKCKVSNKALPAPIEKTISKAKGQPREPQVYTLPPSRDELTKNQVSLTCLVKGFYPSDIAVEWESNGQPENNYKTTPPVLVSDGSFTLASKLTVDKSRWQQGNVFSCSVMHEALHNHYTQKSLSLSPGK

SEQ ID NO: 51 - protein, 232 aa, synthetic construct
EPKSCDKTHTCPPCPAPELLGGPSVFLFPPKPKDTLMISRTPEVTCVVVDVSHEDPEVKFNWYVDGVEVHNAKTKPREEQYNSTYRVVSVLTVLHQDWLNGKEYKCKVSNKALPAPIEKTISKAKGQPREPQVYTLPPSRDKLTKNQVSLTCLVKGFYPSDIAVEWESNGQPENNYKTTPPVLKSDGSFFLASKLTVDKSRWQQGNVFSCSVMHEALHNHYTQKSLSLSPGK

SEQ ID NO: 52 - protein, 232 aa, synthetic construct
EPKSCDKTHTCPPCPAPELLGGPSVFLFPPKPKDTLMISRTPEVTCVVVDVSHEDPEVKFNWYVDGVEVHNAKTKPREEQYNSTYRVVSVLTVLHQDWLNGKEYKCKVSNKALPAPIEKTISKAKGQPREPQVYTLPPSRKELTKNQVSLSCAVKGFYPSDIAVEWESNGQPENNYKTTPPVLDSDGSFFLVSKLTVDKSRWQQGNVFSCSVMHEALHNHYTQKSLSLSPGK

SEQ ID NO: 53 - protein, 232 aa, synthetic construct
EPKSCDKTHTCPPCPAPELLGGPSVFLFPPKPKDTLMISRTPEVTCVVVDVSHEDPEVKFNWYVDGVEVHNAKTKPREEQYNSTYRVVSVLTVLHQDWLNGKEYKCKVSNKALPAPIEKTISKAKGQPREPQVYTLPPSRDDLTKNQVSLSCAVKGFYPSDIAVEWESNGQPENNYKTTPPVLDSDGSFFLVSKLTVDKSRWQQGNVFSCSVMHEALHNHYTQKSLSLSPGK

SEQ ID NO: 54 - protein, 232 aa, synthetic construct
EPKSCDKTHTCPPCPAPELLGGPSVFLFPPKPKDTLMISRTPEVTCVVVDVSHEDPEVKFNWYVDGVEVHNAKTKPREEQYNSTYRVVSVLTVLHQDWLNGKEYKCKVSNKALPAPIEKTISKAKGQPREPRVYTLPPSRDELTKNQVSLSCAVKGFYPSDIAVEWESNGQPENNYKTTPPVLDSDGSFFLVSKLTVDKSRWQQGNVFSCSVMHEALHNHYTQKSLSLSPGK

SEQ ID NO: 55 - protein, 232 aa, synthetic construct
EPKSCDKTHTCPPCPAPELLGGPSVFLFPPKPKDTLMISRTPEVTCVVVDVSHEDPEVKFNWYVDGVEVHNAKTKPREEQYNSTYRVVSVLTVLHQDWLNGKEYKCKVSNKALPAPIEKTISKAKGQPREPQVYTLPPSRKELTKNQVSLTCLVKGFYPSDIAVEWESNGQPENNYKTTPPVLDSDGSFFLASKLTVDKSRWQQGNVFSCSVMHEALHNHYTQKSLSLSPGK

SEQ ID NO: 56 - protein, 232 aa, synthetic construct; identical to SEQ ID NO: 9

SEQ ID NO: 57 - protein, 232 aa, synthetic construct
EPKSCDKTHTCPPCPAPELLGGPSVFLFPPKPKDTLMISRTPEVTCVVVDVSHEDPEVKFNWYVDGVEVHNAKTKPREEQYNSTYRVVSVLTVLHQDWLNGKEYKCKVSNKALPAPIEKTISKAKGQPREPRVYTLPPSRDELTKNQVSLTCLVKGFYPSDIAVEWESNGQPENNYKTTPPVLDSDGSFFLASKLTVDKSRWQQGNVFSCSVMHEALHNHYTQKSLSLSPGK

SEQ ID NO: 58 - protein, 232 aa, synthetic construct
EPKSCDKTHTCPPCPAPELLGGPSVFLFPPKPKDTLMISRTPEVTCVVVDVSHEDPEVKFNWYVDGVEVHNAKTKPREEQYNSTYRVVSVLTVLHQDWLNGKEYKCKVSNKALPAPIEKTISKAKGQPREPQVYTLPPSRDELTKNQVSLTCLVKGFYPSDIAVEWESNGQPENNYKTTPPVLDSDGSFFLYSWLTVDKSRWQQGNVFSCSVMHEALHNHYTQESLSLSPGK

SEQ ID NO: 59 - protein, 232 aa, synthetic construct
EPKSCDKTHTCPPCPAPELLGGPSVFLFPPKPKDTLMISRTPEVTCVVVDVSHEDPEVKFNWYVDGVEVHNAKTKPREEQYNSTYRVVSVLTVLHQDWLNGKEYKCKVSNKALPAPIEKTISKAKGQPREPQVYTLPPSRDELTKNQVSLTCLVEGFYPSDIAVEWESNGQPENNYKTTPPVLDSDGSFFLYSWLTVDKSRWQQGNVFSCSVMHEALHNHYTQKSLSLSPGK

SEQ ID NO: 60 - protein, 232 aa, synthetic construct
EPKSCDKTHTCPPCPAPELLGGPSVFLFPPKPKDTLMISRTPEVTCVVVDVSHEDPEVKFNWYVDGVEVHNAKTKPREEQYNSTYRVVSVLTVLHQDWLNGKEYKCKVSNKALPAPIEKTISKAKGQPREPQVYTLPPSRDELTKNQVSLTCLVYGFYPSDIAVEWESNGQPENNYKTTPPVLDSDGSFFLYSWLTVDKSRWQQGNVFSCSVMHEALHNHYTQKSLSLSPGK

SEQ ID NO: 61 - protein, 232 aa, synthetic construct
EPKSCDKTHTCPPCPAPELLGGPSVFLFPPKPKDTLMISRTPEVTCVVVDVSHEDPEVKFNWYVDGVEVHNAKTKPREEQYNSTYRVVSVLTVLHQDWLNGKEYKCKVSNKALPAPIEKTISKAKGQPREPQVYTLPPSRDELTKNQVSLTCLVYGFYPSDIAVEWESNGQPENNYKTTPPVLDSDGSFFLYSVLTVDKSRWQQGNVFSCSVMHEALHNHYTQESLSLSPGK

SEQ ID NO: 62 - protein, 232 aa, synthetic construct
EPKSCDKTHTCPPCPAPELLGGPSVFLFPPKPKDTLMISRTPEVTCVVVDVSHEDPEVKFNWYVDGVEVHNAKTKPREEQYNSTYRVVSVLTVLHQDWLNGKEYKCKVSNKALPAPIEKTISKAKGQPREPQVYTLPPSRDELTKNQVSLTCLVYGFYPSDIAVEWESNGQPENNYKTTPPVLDSDGSFFLYSDLTVDKSRWQQGNVFSCSVMHEALHNHYTQKSLSLSPGK

SEQ ID NO: 63 - protein, 232 aa, synthetic construct
EPKSCDKTHTCPPCPAPELLGGPSVFLFPPKPKDTLMISRTPEVTCVVVDVSHEDPEVKFNWYVDGVEVHNAKTKPREEQYNSTYRVVSVLTVLHQDWLNGKEYKCKVSNKALPAPIEKTISKAKGQPREPQVYTLPPSRDELTKNQVSLTCLVEGFYPSDIAVEWESNGQPENNYKTTPPVLDSDGSFFLYSWLTVDKSRWQQGNVFSCSVMHEALHNHYTQESLSLSPGK

SEQ ID NO: 64 - protein, 232 aa, synthetic construct
EPKSCDKTHTCPPCPAPELLGGPSVFLFPPKPKDTLMISRTPEVTCVVVDVSHEDPEVKFNWYVDGVEVHNAKTKPREEQYNSTYRVVSVLTVLHQDWLNGKEYKCKVSNKALPAPIEKTISKAKGQPREPQVYTLPPSRDELTKNQVSLTCLVYGFYPSDIAVEWESNGQPENNYKTTPPVLDSDGSFFLYSWLTVDKSRWQQGNVFSCSVMHEALHNHYTQESLSLSPGK

SEQ ID NO: 65 - protein, 232 aa, synthetic construct
EPKSCDKTHTCPPCPAPELLGGPSVFLFPPKPKDTLMISRTPEVTCVVVDVSHEDPEVKFNWYVDGVEVHNAKTKPREEQYNSTYRVVSVLTVLHQDWLNGKEYKCKVSNKALPAPIEKTISKAKGQPREPQVYTLPPSRDELTKNQVSLTCLVYGFYPSDIAVEWESNGQPENNYKTTPPVLDSDGSFFLYSDLTVDKSRWQQGNVFSCSVMHEALHNHYTQESLSLSPGK

SEQ ID NO: 66 - protein, 232 aa, synthetic construct
EPKSCDKTHTCPPCPAPELLGGPSVFLFPPKPKDTLMISRTPEVTCVVVDVSHEDPEVKFNWYVDGVEVHNAKTKPREEQYNSTYRVVSVLTVLHQDWLNGKEYKCKVSNKALPAPIEKTISKAKGQPREPQVYTLPPSRDELTDNQVSLTCLVKGFYPSDIAVEWESNGQPENNYKTTPPVLDSDGSFFLYSVLTVDKSRWQQGNVFSCSVMHEALHNHYTQESLSLSPGK

SEQ ID NO: 67 - protein, 232 aa, synthetic construct
EPKSCDKTHTCPPCPAPELLGGPSVFLFPPKPKDTLMISRTPEVTCVVVDVSHEDPEVKFNWYVDGVEVHNAKTKPREEQYNSTYRVVSVLTVLHQDWLNGKEYKCKVSNKALPAPIEKTISKAKGQPREPQVYTLPPSRDELTDNQVSLTCLVEGFYPSDIAVEWESNGQPENNYKTTPPVLDSDGSFFLYSVLTVDKSRWQQGNVFSCSVMHEALHNHYTQKSLSLSPGK

SEQ ID NO: 68 - protein, 232 aa, synthetic construct
EPKSCDKTHTCPPCPAPELLGGPSVFLFPPKPKDTLMISRTPEVTCVVVDVSHEDPEVKFNWYVDGVEVHNAKTKPREEQYNSTYRVVSVLTVLHQDWLNGKEYKCKVSNKALPAPIEKTISKAKGQPREPQVYTLPPSRDELTDNQVSLTCLVKGFYPSDIAVEWESNGQPENNYKTTPPVLDSDGSFFLYSDLTVDKSRWQQGNVFSCSVMHEALHNHYTQKSLSLSPGK

SEQ ID NO: 69 - protein, 232 aa, synthetic construct
EPKSCDKTHTCPPCPAPELLGGPSVFLFPPKPKDTLMISRTPEVTCVVVDVSHEDPEVKFNWYVDGVEVHNAKTKPREEQYNSTYRVVSVLTVLHQDWLNGKEYKCKVSNKALPAPIEKTISKAKGQPREPQVYTLPPSRDELTDNQVSLTCLVYGFYPSDIAVEWESNGQPENNYKTTPPVLDSDGSFFLYSVLTVDKSRWQQGNVFSCSVMHEALHNHYTQKSLSLSPGK

SEQ ID NO: 70 - protein, 232 aa, synthetic construct
EPKSCDKTHTCPPCPAPELLGGPSVFLFPPKPKDTLMISRTPEVTCVVVDVSHEDPEVKFNWYVDGVEVHNAKTKPREEQYNSTYRVVSVLTVLHQDWLNGKEYKCKVSNKALPAPIEKTISKAKGQPREPQVYTLPPSRDELTKNQVSLTCLVKGFYPSDIAVEWESNGQPENNYKTTPPVLDSDGSFFLKSKLTVDKSRWQQGNVFSCSVMHEALHNHYTQKSLSLSPGK

SEQ ID NO: 71 - protein, 232 aa, synthetic construct
EPKSCDKTHTCPPCPAPELLGGPSVFLFPPKPKDTLMISRTPEVTCVVVDVSHEDPEVKFNWYVDGVEVHNAKTKPREEQYNSTYRVVSVLTVLHQDWLNGKEYKCKVSNKALPAPIEKTISKAKGQPREPQVYTLPPSRDELTKNQVSLTCLVKGFYPSDIAVEWESNGQPENNYKTTPPVLDSDGSFFLYSKLTVDKSRWQQGNVFSCSVMHEALHNHYTQWSLSLSPGK

SEQ ID NO: 72 - protein, 232 aa, synthetic construct
EPKSCDKTHTCPPCPAPELLGGPSVFLFPPKPKDTLMISRTPEVTCVVVDVSHEDPEVKFNWYVDGVEVHNAKTKPREEQYNSTYRVVSVLTVLHQDWLNGKEYKCKVSNKALPAPIEKTISKAKGQPREPQVYTLPPSRDELTKNQVSLTCLVWGFYPSDIAVEWESNGQPENNYKTTPPVLDSDGSFFLYSKLTVDKSRWQQGNVFSCSVMHEALHNHYTQKSLSLSPGK

SEQ ID NO: 73 - protein, 232 aa, synthetic construct
EPKSCDKTHTCPPCPAPELLGGPSVFLFPPKPKDTLMISRTPEVTCVVVDVSHEDPEVKFNWYVDGVEVHNAKTKPREEQYNSTYRVVSVLTVLHQDWLNGKEYKCKVSNKALPAPIEKTISKAKGQPREPQVYTLPPSRDELTKNQVSLTCLVKGFYPSDIAVEWESNGQPENNYKTSPPALDSDGSFALVSKLTVDKSRWQQGNVFSCSVMHEALHNHYTQKSLSLSPGK

SEQ ID NO: 74 - protein, 232 aa, synthetic construct
EPKSCDKTHTCPPCPAPELLGGPSVFLFPPKPKDTLMISRTPEVTCVVVDVSHEDPEVKFNWYVDGVEVHNAKTKPREEQYNSTYRVVSVLTVLHQDWLNGKEYKCKVSNKALPAPIEKTISKAKGQPREPQVYTLPPSRDELTWNQVSLTCLVKGFYPSDIAVEWESNGQPENNYKTTPPVLDSDGSFFLYSKLTVDKSRWQQGNVFSCSVMHEALHNHYTQKSLSLSPGK

SEQ ID NO: 75 - DNA, 696 bp, synthetic construct
  source 1..696: mol_type = other DNA
gagcccaagagctgcgacaagacccacacctgccccccctgccccgcccccgagctgctgggcggccccagcgtgttcctgttcccccccaagcccaaggacaccctgatgatcagcaggacccccgaggtgacctgcgtggtggtggacgtgagccacgaggaccccgaggtgaagttcaactggtacgtggacggcgtggaggtgcacaacgccaagaccaagcccagggaggagcagtacaacagcacctacagggtggtgagcgtgctgaccgtgctgcaccaggactggctgaacggcaaggagtacaagtgcaaggtgagcaacaaggccctgcccgcccccatcgagaagaccatcagcaaggccaagggccagcccagggagccccaggtgtacaccctgccccccagcagggacgagctgaccaagaaccaggtgagcctgtggtgcctggtgaagggcttctaccccagcgacatcgccgtggagtgggagagcaacggccagcccgagaacaactacaagaccaccccccccgtgctggtgagcgacggcagcttcaccctgtacagcaagctgaccgtggacaagagcaggtggcagcagggcaacgtgttcagctgcagcgtgatgcacgaggccctgcacaaccactacacccagaagagcctgagcctgagccccggcaag

SEQ ID NO: 76 - DNA, 696 bp, synthetic construct
  source 1..696: mol_type = other DNA
gagcccaagagctgcgacaagacccacacctgccccccctgccccgcccccgagctgctgggcggccccagcgtgttcctgttcccccccaagcccaaggacaccctgatgatcagcaggacccccgaggtgacctgcgtggtggtggacgtgagccacgaggaccccgaggtgaagttcaactggtacgtggacggcgtggaggtgcacaacgccaagaccaagcccagggaggagcagtacaacagcacctacagggtggtgagcgtgctgaccgtgctgcaccaggactggctgaacggcaaggagtacaagtgcaaggtgagcaacaaggccctgcccgcccccatcgagaagaccatcagcaaggccaagggccagcccagggagccccaggtgtacaccctgccccccagcagggacaagctgaccaagaaccaggtgagcctgtggtgcctggtgaagggcttctaccccagcgacatcgccgtggagtgggagagcaacggccagcccgagaacaactacaagaccaccccccccgtgctgaagagcgacggcagcttcttcctgtacagcaagctgaccgtggacaagagcaggtggcagcagggcaacgtgttcagctgcagcgtgatgcacgaggccctgcacaaccactacacccagaagagcctgagcctgagccccggcaag

SEQ ID NO: 77 - DNA, 696 bp, synthetic construct
  source 1..696: mol_type = other DNA
gagcccaagagctgcgacaagacccacacctgccccccctgccccgcccccgagctgctgggcggccccagcgtgttcctgttcccccccaagcccaaggacaccctgatgatcagcaggacccccgaggtgacctgcgtggtggtggacgtgagccacgaggaccccgaggtgaagttcaactggtacgtggacggcgtggaggtgcacaacgccaagaccaagcccagggaggagcagtacaacagcacctacagggtggtgagcgtgctgaccgtgctgcaccaggactggctgaacggcaaggagtacaagtgcaaggtgagcaacaaggccctgcccgcccccatcgagaagaccatcagcaaggccaagggccagcccagggagccccaggtgtacaccctgccccccagcagggacgagctgaccaagaaccaggtgagcctggtgtgcctggtgaagggcttctaccccagcgacatcgccgtggagtgggagagcaacggccagcccgagaacaactacaagaccaccccccccgtgctggtgagcgacggcagcttcaccctgtacagcaagctgaccgtggacaagagcaggtggcagcagggcaacgtgttcagctgcagcgtgatgcacgaggccctgcacaaccactacacccagaagagcctgagcctgagccccggcaag

SEQ ID NO: 78 - DNA, 696 bp, synthetic construct
  source 1..696: mol_type = other DNA
gagcccaagagctgcgacaagacccacacctgccccccctgccccgcccccgagctgctgggcggccccagcgtgttcctgttcccccccaagcccaaggacaccctgatgatcagcaggacccccgaggtgacctgcgtggtggtggacgtgagccacgaggaccccgaggtgaagttcaactggtacgtggacggcgtggaggtgcacaacgccaagaccaagcccagggaggagcagtacaacagcacctacagggtggtgagcgtgctgaccgtgctgcaccaggactggctgaacggcaaggagtacaagtgcaaggtgagcaacaaggccctgcccgcccccatcgagaagaccatcagcaaggccaagggccagcccagggagccccaggtgtacaccctgccccccagcagggacaagctgaccaagaaccaggtgagcctggtgtgcctggtgaagggcttctaccccagcgacatcgccgtggagtgggagagcaacggccagcccgagaacaactacaagaccaccccccccgtgctgaagagcgacggcagcttcttcctgtacagcaagctgaccgtggacaagagcaggtggcagcagggcaacgtgttcagctgcagcgtgatgcacgaggccctgcacaaccactacacccagaagagcctgagcctgagccccggcaag

SEQ ID NO: 79 - DNA, 696 bp, synthetic construct
  source 1..696: mol_type = other DNA
gagcccaagagctgcgacaagacccacacctgccccccctgccccgcccccgagctgctgggcggccccagcgtgttcctgttcccccccaagcccaaggacaccctgatgatcagcaggacccccgaggtgacctgcgtggtggtggacgtgagccacgaggaccccgaggtgaagttcaactggtacgtggacggcgtggaggtgcacaacgccaagaccaagcccagggaggagcagtacaacagcacctacagggtggtgagcgtgctgaccgtgctgcaccaggactggctgaacggcaaggagtacaagtgcaaggtgagcaacaaggccctgcccgcccccatcgagaagaccatcagcaaggccaagggccagcccagggagccccaggtgtacaccctgccccccagcaggaaggagctgaccaagaaccaggtgagcctgtggtgcctggtgaagggcttctaccccagcgacatcgccgtggagtgggagagcaacggccagcccgagaacaactacaagaccaccccccccgtgctggacagcgacggcagcttcttcctgtacagcaagctgaccgtggacaagagcaggtggcagcagggcaacgtgttcagctgcagcgtgatgcacgaggccctgcacaaccactacacccagaagagcctgagcctgagccccggcaag

SEQ ID NO: 80 - DNA, 696 bp, synthetic construct
  source 1..696: mol_type = other DNA
gagcccaagagctgcgacaagacccacacctgccccccctgccccgcccccgagctgctgggcggccccagcgtgttcctgttcccccccaagcccaaggacaccctgatgatcagcaggacccccgaggtgacctgcgtggtggtggacgtgagccacgaggaccccgaggtgaagttcaactggtacgtggacggcgtggaggtgcacaacgccaagaccaagcccagggaggagcagtacaacagcacctacagggtggtgagcgtgctgaccgtgctgcaccaggactggctgaacggcaaggagtacaagtgcaaggtgagcaacaaggccctgcccgcccccatcgagaagaccatcagcaaggccaagggccagcccagggagccccaggtgtacaccctgccccccagcagggacgacctgaccaagaaccaggtgagcctgtggtgcctggtgaagggcttctaccccagcgacatcgccgtggagtgggagagcaacggccagcccgagaacaactacaagaccaccccccccgtgctggacagcgacggcagcttcttcctgtacagcaagctgaccgtggacaagagcaggtggcagcagggcaacgtgttcagctgcagcgtgatgcacgaggccctgcacaaccactacacccagaagagcctgagcctgagccccggcaag

SEQ ID NO: 81 - DNA, 696 bp, synthetic construct
  source 1..696: mol_type = other DNA
gagcccaagagctgcgacaagacccacacctgccccccctgccccgcccccgagctgctgggcggccccagcgtgttcctgttcccccccaagcccaaggacaccctgatgatcagcaggacccccgaggtgacctgcgtggtggtggacgtgagccacgaggaccccgaggtgaagttcaactggtacgtggacggcgtggaggtgcacaacgccaagaccaagcccagggaggagcagtacaacagcacctacagggtggtgagcgtgctgaccgtgctgcaccaggactggctgaacggcaaggagtacaagtgcaaggtgagcaacaaggccctgcccgcccccatcgagaagaccatcagcaaggccaagggccagcccagggagcccagggtgtacaccctgccccccagcagggacgagctgaccaagaaccaggtgagcctgtggtgcctggtgaagggcttctaccccagcgacatcgccgtggagtgggagagcaacggccagcccgagaacaactacaagaccaccccccccgtgctggacagcgacggcagcttcttcctgtacagcaagctgaccgtggacaagagcaggtggcagcagggcaacgtgttcagctgcagcgtgatgcacgaggccctgcacaaccactacacccagaagagcctgagcctgagccccggcaag

SEQ ID NO: 82 - DNA, 696 bp, synthetic construct
  source 1..696: mol_type = other DNA
gagcccaagagctgcgacaagacccacacctgccccccctgccccgcccccgagctgctgggcggccccagcgtgttcctgttcccccccaagcccaaggacaccctgatgatcagcaggacccccgaggtgacctgcgtggtggtggacgtgagccacgaggaccccgaggtgaagttcaactggtacgtggacggcgtggaggtgcacaacgccaagaccaagcccagggaggagcagtacaacagcacctacagggtggtgagcgtgctgaccgtgctgcaccaggactggctgaacggcaaggagtacaagtgcaaggtgagcaacaaggccctgcccgcccccatcgagaagaccatcagcaaggccaagggccagcccagggagccccaggtgtacaccctgccccccagcaggaaggagctgaccaagaaccaggtgagcctggtgtgcctggtgaagggcttctaccccagcgacatcgccgtggagtgggagagcaacggccagcccgagaacaactacaagaccaccccccccgtgctggacagcgacggcagcttcttcctgtacagcaagctgaccgtggacaagagcaggtggcagcagggcaacgtgttcagctgcagcgtgatgcacgaggccctgcacaaccactacacccagaagagcctgagcctgagccccggcaag

SEQ ID NO: 83 - DNA, 696 bp, synthetic construct
  source 1..696: mol_type = other DNA
gagcccaagagctgcgacaagacccacacctgccccccctgccccgcccccgagctgctgggcggccccagcgtgttcctgttcccccccaagcccaaggacaccctgatgatcagcaggacccccgaggtgacctgcgtggtggtggacgtgagccacgaggaccccgaggtgaagttcaactggtacgtggacggcgtggaggtgcacaacgccaagaccaagcccagggaggagcagtacaacagcacctacagggtggtgagcgtgctgaccgtgctgcaccaggactggctgaacggcaaggagtacaagtgcaaggtgagcaacaaggccctgcccgcccccatcgagaagaccatcagcaaggccaagggccagcccagggagccccaggtgtacaccctgccccccagcagggacgacctgaccaagaaccaggtgagcctggtgtgcctggtgaagggcttctaccccagcgacatcgccgtggagtgggagagcaacggccagcccgagaacaactacaagaccaccccccccgtgctggacagcgacggcagcttcttcctgtacagcaagctgaccgtggacaagagcaggtggcagcagggcaacgtgttcagctgcagcgtgatgcacgaggccctgcacaaccactacacccagaagagcctgagcctgagccccggcaag

SEQ ID NO: 84 - DNA, 696 bp, synthetic construct
  source 1..696: mol_type = other DNA
gagcccaagagctgcgacaagacccacacctgccccccctgccccgcccccgagctgctgggcggccccagcgtgttcctgttcccccccaagcccaaggacaccctgatgatcagcaggacccccgaggtgacctgcgtggtggtggacgtgagccacgaggaccccgaggtgaagttcaactggtacgtggacggcgtggaggtgcacaacgccaagaccaagcccagggaggagcagtacaacagcacctacagggtggtgagcgtgctgaccgtgctgcaccaggactggctgaacggcaaggagtacaagtgcaaggtgagcaacaaggccctgcccgcccccatcgagaagaccatcagcaaggccaagggccagcccagggagcccagggtgtacaccctgccccccagcagggacgagctgaccaagaaccaggtgagcctggtgtgcctggtgaagggcttctaccccagcgacatcgccgtggagtgggagagcaacggccagcccgagaacaactacaagaccaccccccccgtgctggacagcgacggcagcttcttcctgtacagcaagctgaccgtggacaagagcaggtggcagcagggcaacgtgttcagctgcagcgtgatgcacgaggccctgcacaaccactacacccagaagagcctgagcctgagccccggcaag

SEQ ID NO: 85 - DNA, 696 bp, synthetic construct
  source 1..696: mol_type = other DNA
gagcccaagagctgcgacaagacccacacctgccccccctgccccgcccccgagctgctgggcggccccagcgtgttcctgttcccccccaagcccaaggacaccctgatgatcagcaggacccccgaggtgacctgcgtggtggtggacgtgagccacgaggaccccgaggtgaagttcaactggtacgtggacggcgtggaggtgcacaacgccaagaccaagcccagggaggagcagtacaacagcacctacagggtggtgagcgtgctgaccgtgctgcaccaggactggctgaacggcaaggagtacaagtgcaaggtgagcaacaaggccctgcccgcccccatcgagaagaccatcagcaaggccaagggccagcccagggagccccaggtgtacaccctgccccccagcagggacgagctgaccaagaaccaggtgagcctgtggtgcctggtgaagggcttctaccccagcgacatcgccgtggagtgggagagcaacggccagcccgagaacaactacaagaccaccccccccgtgctggacagcgacggcagcttcttcctgtacagctggctgaccgtggacaagagcaggtggcagcagggcaacgtgttcagctgcagcgtgatgcacgaggccctgcacaaccactacacccagaagagcctgagcctgagccccggcaag

SEQ ID NO: 86 - DNA, 696 bp, synthetic construct
  source 1..696: mol_type = other DNA
gagcccaagagctgcgacaagacccacacctgccccccctgccccgcccccgagctgctgggcggccccagcgtgttcctgttcccccccaagcccaaggacaccctgatgatcagcaggacccccgaggtgacctgcgtggtggtggacgtgagccacgaggaccccgaggtgaagttcaactggtacgtggacggcgtggaggtgcacaacgccaagaccaagcccagggaggagcagtacaacagcacctacagggtggtgagcgtgctgaccgtgctgcaccaggactggctgaacggcaaggagtacaagtgcaaggtgagcaacaaggccctgcccgcccccatcgagaagaccatcagcaaggccaagggccagcccagggagccccaggtgtacaccctgccccccagcagggacgagctgaccaagaaccaggtgagcctgtggtgcctggtggagggcttctaccccagcgacatcgccgtggagtgggagagcaacggccagcccgagaacaactacaagaccaccccccccgtgctggacagcgacggcagcttcttcctgtacagcgacctgaccgtggacaagagcaggtggcagcagggcaacgtgttcagctgcagcgtgatgcacgaggccctgcacaaccactacacccagaagagcctgagcctgagccccggcaag

SEQ ID NO: 87 - DNA, 696 bp, synthetic construct
  source 1..696: mol_type = other DNA
gagcccaagagctgcgacaagacccacacctgccccccctgccccgcccccgagctgctgggcggccccagcgtgttcctgttcccccccaagcccaaggacaccctgatgatcagcaggacccccgaggtgacctgcgtggtggtggacgtgagccacgaggaccccgaggtgaagttcaactggtacgtggacggcgtggaggtgcacaacgccaagaccaagcccagggaggagcagtacaacagcacctacagggtggtgagcgtgctgaccgtgctgcaccaggactggctgaacggcaaggagtacaagtgcaaggtgagcaacaaggccctgcccgcccccatcgagaagaccatcagcaaggccaagggccagcccagggagccccaggtgtacaccctgccccccagcagggacgagctgaccaagaaccaggtgagcctggtgtgcctggtgaagggcttctaccccagcgacatcgccgtggagtgggagagcaacggccagcccgagaacaactacaagaccaccccccccgtgctggacagcgacggcagcttcttcctgtacagctggctgaccgtggacaagagcaggtggcagcagggcaacgtgttcagctgcagcgtgatgcacgaggccctgcacaaccactacacccagaagagcctgagcctgagccccggcaag

SEQ ID NO: 88 - DNA, 696 bp, synthetic construct
  source 1..696: mol_type = other DNA
gagcccaagagctgcgacaagacccacacctgccccccctgccccgcccccgagctgctgggcggccccagcgtgttcctgttcccccccaagcccaaggacaccctgatgatcagcaggacccccgaggtgacctgcgtggtggtggacgtgagccacgaggaccccgaggtgaagttcaactggtacgtggacggcgtggaggtgcacaacgccaagaccaagcccagggaggagcagtacaacagcacctacagggtggtgagcgtgctgaccgtgctgcaccaggactggctgaacggcaaggagtacaagtgcaaggtgagcaacaaggccctgcccgcccccatcgagaagaccatcagcaaggccaagggccagcccagggagccccaggtgtacaccctgccccccagcagggacgagctgaccaagaaccaggtgagcctggtgtgcctggtggagggcttctaccccagcgacatcgccgtggagtgggagagcaacggccagcccgagaacaactacaagaccaccccccccgtgctggacagcgacggcagcttcttcctgtacagcgacctgaccgtggacaagagcaggtggcagcagggcaacgtgttcagctgcagcgtgatgcacgaggccctgcacaaccactacacccagaagagcctgagcctgagccccggcaag

SEQ ID NO: 89 - DNA, 696 bp, synthetic construct
  source 1..696: mol_type = other DNA
gagcccaagagctgcgacaagacccacacctgccccccctgccccgcccccgagctgctgggcggccccagcgtgttcctgttcccccccaagcccaaggacaccctgatgatcagcaggacccccgaggtgacctgcgtggtggtggacgtgagccacgaggaccccgaggtgaagttcaactggtacgtggacggcgtggaggtgcacaacgccaagaccaagcccagggaggagcagtacaacagcacctacagggtggtgagcgtgctgaccgtgctgcaccaggactggctgaacggcaaggagtacaagtgcaaggtgagcaacaaggccctgcccgcccccatcgagaagaccatcagcaaggccaagggccagcccagggagccccaggtgtacaccctgccccccagcagggacgagctgaccaagaaccaggtgagcctgtggtgcctggtgaagggcttctaccccagcgacatcgccgtggagtgggagagcaacggccagcccgagaacaactacaagaccaccccccccgtgctggacagcgacggcagcttcttcctgtacagcaagctgaccgtggacaagagcaggtggcagcagggcaacgtgttcagctgcagcgtgatgcacgaggccctgcacaaccactacacccaggagagcctgagcctgagccccggcaag

SEQ ID NO: 90 - DNA, 696 bp, synthetic construct
  source 1..696: mol_type = other DNA
gagcccaagagctgcgacaagacccacacctgccccccctgccccgcccccgagctgctgggcggccccagcgtgttcctgttcccccccaagcccaaggacaccctgatgatcagcaggacccccgaggtgacctgcgtggtggtggacgtgagccacgaggaccccgaggtgaagttcaactggtacgtggacggcgtggaggtgcacaacgccaagaccaagcccagggaggagcagtacaacagcacctacagggtggtgagcgtgctgaccgtgctgcaccaggactggctgaacggcaaggagtacaagtgcaaggtgagcaacaaggccctgcccgcccccatcgagaagaccatcagcaaggccaagggccagcccagggagccccaggtgtacaccctgccccccagcagggacgagctgaccaagaaccaggtgagcctgtggtgcctggtgtacggcttctaccccagcgacatcgccgtggagtgggagagcaacggccagcccgagaacaactacaagaccaccccccccgtgctggacagcgacggcagcttcttcctgtacagcaagctgaccgtggacaagagcaggtggcagcagggcaacgtgttcagctgcagcgtgatgcacgaggccctgcacaaccactacacccagaagagcctgagcctgagccccggcaag

SEQ ID NO: 91 - DNA, 696 bp, synthetic construct
  source 1..696: mol_type = other DNA
gagcccaagagctgcgacaagacccacacctgccccccctgccccgcccccgagctgctgggcggccccagcgtgttcctgttcccccccaagcccaaggacaccctgatgatcagcaggacccccgaggtgacctgcgtggtggtggacgtgagccacgaggaccccgaggtgaagttcaactggtacgtggacggcgtggaggtgcacaacgccaagaccaagcccagggaggagcagtacaacagcacctacagggtggtgagcgtgctgaccgtgctgcaccaggactggctgaacggcaaggagtacaagtgcaaggtgagcaacaaggccctgcccgcccccatcgagaagaccatcagcaaggccaagggccagcccagggagccccaggtgtacaccctgccccccagcagggacgagctgaccgacaaccaggtgagcctgtggtgcctggtgaagggcttctaccccagcgacatcgccgtggagtgggagagcaacggccagcccgagaacaactacaagaccaccccccccgtgctggacagcgacggcagcttcttcctgtacagcaagctgaccgtggacaagagcaggtggcagcagggcaacgtgttcagctgcagcgtgatgcacgaggccctgcacaaccactacacccagaagagcctgagcctgagccccggcaag

SEQ ID NO: 92 - DNA, 696 bp, synthetic construct
  source 1..696: mol_type = other DNA
gagcccaagagctgcgacaagacccacacctgccccccctgccccgcccccgagctgctgggcggccccagcgtgttcctgttcccccccaagcccaaggacaccctgatgatcagcaggacccccgaggtgacctgcgtggtggtggacgtgagccacgaggaccccgaggtgaagttcaactggtacgtggacggcgtggaggtgcacaacgccaagaccaagcccagggaggagcagtacaacagcacctacagggtggtgagcgtgctgaccgtgctgcaccaggactggctgaacggcaaggagtacaagtgcaaggtgagcaacaaggccctgcccgcccccatcgagaagaccatcagcaaggccaagggccagcccagggagccccaggtgtacaccctgccccccagcagggacgagctgaccaagaaccaggtgagcctggtgtgcctggtgaagggcttctaccccagcgacatcgccgtggagtgggagagcaacggccagcccgagaacaactacaagaccaccccccccgtgctggacagcgacggcagcttcttcctgtacagcaagctgaccgtggacaagagcaggtggcagcagggcaacgtgttcagctgcagcgtgatgcacgaggccctgcacaaccactacacccaggagagcctgagcctgagccccggcaag

SEQ ID NO: 93 - DNA, 696 bp, synthetic construct
  source 1..696: mol_type = other DNA
gagcccaagagctgcgacaagacccacacctgccccccctgccccgcccccgagctgctgggcggccccagcgtgttcctgttcccccccaagcccaaggacaccctgatgatcagcaggacccccgaggtgacctgcgtggtggtggacgtgagccacgaggaccccgaggtgaagttcaactggtacgtggacggcgtggaggtgcacaacgccaagaccaagcccagggaggagcagtacaacagcacctacagggtggtgagcgtgctgaccgtgctgcaccaggactggctgaacggcaaggagtacaagtgcaaggtgagcaacaaggccctgcccgcccccatcgagaagaccatcagcaaggccaagggccagcccagggagccccaggtgtacaccctgccccccagcagggacgagctgaccaagaaccaggtgagcctgacctgcctggtgtacggcttctaccccagcgacatcgccgtggagtgggagagcaacggccagcccgagaacaactacaagaccaccccccccgtgctggacagcgacggcagcttcttcctggccagcaagctgaccgtggacaagagcaggtggcagcagggcaacgtgttcagctgcagcgtgatgcacgaggccctgcacaaccactacacccagaagagcctgagcctgagccccggcaag

SEQ ID NO: 94 - DNA, 696 bp, synthetic construct
  source 1..696: mol_type = other DNA
gagcccaagagctgcgacaagacccacacctgccccccctgccccgcccccgagctgctgggcggccccagcgtgttcctgttcccccccaagcccaaggacaccctgatgatcagcaggacccccgaggtgacctgcgtggtggtggacgtgagccacgaggaccccgaggtgaagttcaactggtacgtggacggcgtggaggtgcacaacgccaagaccaagcccagggaggagcagtacaacagcacctacagggtggtgagcgtgctgaccgtgctgcaccaggactggctgaacggcaaggagtacaagtgcaaggtgagcaacaaggccctgcccgcccccatcgagaagaccatcagcaaggccaagggccagcccagggagccccaggtgtacaccctgccccccagcagggacgagctgaccgacaaccaggtgagcctggtgtgcctggtgaagggcttctaccccagcgacatcgccgtggagtgggagagcaacggccagcccgagaacaactacaagaccaccccccccgtgctggacagcgacggcagcttcttcctgtacagcaagctgaccgtggacaagagcaggtggcagcagggcaacgtgttcagctgcagcgtgatgcacgaggccctgcacaaccactacacccagaagagcctgagcctgagccccggcaag

SEQ ID NO: 95 - DNA, 696 bp, synthetic construct
  source 1..696: mol_type = other DNA
gagcccaagagctgcgacaagacccacacctgccccccctgccccgcccccgagctgctgggcggccccagcgtgttcctgttcccccccaagcccaaggacaccctgatgatcagcaggacccccgaggtgacctgcgtggtggtggacgtgagccacgaggaccccgaggtgaagttcaactggtacgtggacggcgtggaggtgcacaacgccaagaccaagcccagggaggagcagtacaacagcacctacagggtggtgagcgtgctgaccgtgctgcaccaggactggctgaacggcaaggagtacaagtgcaaggtgagcaacaaggccctgcccgcccccatcgagaagaccatcagcaaggccaagggccagcccagggagccccaggtgtacaccctgccccccagcaggaaggagctgaccaagaaccaggtgagcctgacctgcctggtgaagggcttctaccccagcgacatcgccgtggagtgggagagcaacggccagcccgagaacaactacaagaccaccccccccgtgctggtgagcgacggcagcttcaccctgtacagcaagctgaccgtggacaagagcaggtggcagcagggcaacgtgttcagctgcagcgtgatgcacgaggccctgcacaaccactacacccagaagagcctgagcctgagccccggcaag

SEQ ID NO: 96 - DNA, 696 bp, synthetic construct
  source 1..696: mol_type = other DNA
gagcccaagagctgcgacaagacccacacctgccccccctgccccgcccccgagctgctgggcggccccagcgtgttcctgttcccccccaagcccaaggacaccctgatgatcagcaggacccccgaggtgacctgcgtggtggtggacgtgagccacgaggaccccgaggtgaagttcaactggtacgtggacggcgtggaggtgcacaacgccaagaccaagcccagggaggagcagtacaacagcacctacagggtggtgagcgtgctgaccgtgctgcaccaggactggctgaacggcaaggagtacaagtgcaaggtgagcaacaaggccctgcccgcccccatcgagaagaccatcagcaaggccaagggccagcccagggagccccaggtgtacaccctgccccccagcagggacaagctgaccaagaaccaggtgagcctgacctgcctggtgaagggcttctaccccagcgacatcgccgtggagtgggagagcaacggccagcccgagaacaactacaagaccaccccccccgtgctggtgagcgacggcagcttcaccctgtacagcaagctgaccgtggacaagagcaggtggcagcagggcaacgtgttcagctgcagcgtgatgcacgaggccctgcacaaccactacacccagaagagcctgagcctgagccccggcaag

SEQ ID NO: 97 - DNA, 696 bp, synthetic construct
  source 1..696: mol_type = other DNA
gagcccaagagctgcgacaagacccacacctgccccccctgccccgcccccgagctgctgggcggccccagcgtgttcctgttcccccccaagcccaaggacaccctgatgatcagcaggacccccgaggtgacctgcgtggtggtggacgtgagccacgaggaccccgaggtgaagttcaactggtacgtggacggcgtggaggtgcacaacgccaagaccaagcccagggaggagcagtacaacagcacctacagggtggtgagcgtgctgaccgtgctgcaccaggactggctgaacggcaaggagtacaagtgcaaggtgagcaacaaggccctgcccgcccccatcgagaagaccatcagcaaggccaagggccagcccagggagccccaggtgtacaccctgccccccagcagggacgacctgaccaagaaccaggtgagcctgacctgcctggtgaagggcttctaccccagcgacatcgccgtggagtgggagagcaacggccagcccgagaacaactacaagaccaccccccccgtgctggtgagcgacggcagcttcaccctgtacagcaagctgaccgtggacaagagcaggtggcagcagggcaacgtgttcagctgcagcgtgatgcacgaggccctgcacaaccactacacccagaagagcctgagcctgagccccggcaag

SEQ ID NO: 98 - DNA, 696 bp, synthetic construct
  source 1..696: mol_type = other DNA
gagcccaagagctgcgacaagacccacacctgccccccctgccccgcccccgagctgctgggcggccccagcgtgttcctgttcccccccaagcccaaggacaccctgatgatcagcaggacccccgaggtgacctgcgtggtggtggacgtgagccacgaggaccccgaggtgaagttcaactggtacgtggacggcgtggaggtgcacaacgccaagaccaagcccagggaggagcagtacaacagcacctacagggtggtgagcgtgctgaccgtgctgcaccaggactggctgaacggcaaggagtacaagtgcaaggtgagcaacaaggccctgcccgcccccatcgagaagaccatcagcaaggccaagggccagcccagggagccccaggtgtacaccctgccccccagcaggaaggacctgaccaagaaccaggtgagcctgacctgcctggtgaagggcttctaccccagcgacatcgccgtggagtgggagagcaacggccagcccgagaacaactacaagaccaccccccccgtgctggacagcgacggcagcttcttcctggccagcaagctgaccgtggacaagagcaggtggcagcagggcaacgtgttcagctgcagcgtgatgcacgaggccctgcacaaccactacacccagaagagcctgagcctgagccccggcaag

SEQ ID NO: 99 - DNA, 696 bp, synthetic construct
  source 1..696: mol_type = other DNA
gagcccaagagctgcgacaagacccacacctgccccccctgccccgcccccgagctgctgggcggccccagcgtgttcctgttcccccccaagcccaaggacaccctgatgatcagcaggacccccgaggtgacctgcgtggtggtggacgtgagccacgaggaccccgaggtgaagttcaactggtacgtggacggcgtggaggtgcacaacgccaagaccaagcccagggaggagcagtacaacagcacctacagggtggtgagcgtgctgaccgtgctgcaccaggactggctgaacggcaaggagtacaagtgcaaggtgagcaacaaggccctgcccgcccccatcgagaagaccatcagcaaggccaagggccagcccagggagccccaggtgtacaccctgccccccagcagggacgacctgaccaagaaccaggtgagcctgacctgcctggtgaagggcttctaccccagcgacatcgccgtggagtgggagagcaacggccagcccgagaacaactacaagaccaccccccccgtgctgaagagcgacggcagcttcttcctgtacagcaagctgaccgtggacaagagcaggtggcagcagggcaacgtgttcagctgcagcgtgatgcacgaggccctgcacaaccactacacccagaagagcctgagcctgagccccggcaag

SEQ ID NO: 100 - DNA, 696 bp, synthetic construct
  source 1..696: mol_type = other DNA
gagcccaagagctgcgacaagacccacacctgccccccctgccccgcccccgagctgctgggcggccccagcgtgttcctgttcccccccaagcccaaggacaccctgatgatcagcaggacccccgaggtgacctgcgtggtggtggacgtgagccacgaggaccccgaggtgaagttcaactggtacgtggacggcgtggaggtgcacaacgccaagaccaagcccagggaggagcagtacaacagcacctacagggtggtgagcgtgctgaccgtgctgcaccaggactggctgaacggcaaggagtacaagtgcaaggtgagcaacaaggccctgcccgcccccatcgagaagaccatcagcaaggccaagggccagcccagggagccccaggtgtacaccctgccccccagcaggaagaagctgaccaagaaccaggtgagcctgacctgcctggtgaagggcttctaccccagcgacatcgccgtggagtgggagagcaacggccagcccgagaacaactacaagaccaccccccccgtgctggtgagcgacggcagcttcaccctgtacagcaagctgaccgtggacaagagcaggtggcagcagggcaacgtgttcagctgcagcgtgatgcacgaggccctgcacaaccactacacccagaagagcctgagcctgagccccggcaag

SEQ ID NO: 101 - DNA, 696 bp, synthetic construct
  source 1..696: mol_type = other DNA
gagcccaagagctgcgacaagacccacacctgccccccctgccccgcccccgagctgctgggcggccccagcgtgttcctgttcccccccaagcccaaggacaccctgatgatcagcaggacccccgaggtgacctgcgtggtggtggacgtgagccacgaggaccccgaggtgaagttcaactggtacgtggacggcgtggaggtgcacaacgccaagaccaagcccagggaggagcagtacaacagcacctacagggtggtgagcgtgctgaccgtgctgcaccaggactggctgaacggcaaggagtacaagtgcaaggtgagcaacaaggccctgcccgcccccatcgagaagaccatcagcaaggccaagggccagcccagggagccccaggtgtacaccctgccccccagcaggaaggacctgaccaagaaccaggtgagcctgacctgcctggtgaagggcttctaccccagcgacatcgccgtggagtgggagagcaacggccagcccgagaacaactacaagaccaccccccccgtgctggtgagcgacggcagcttcaccctgtacagcaagctgaccgtggacaagagcaggtggcagcagggcaacgtgttcagctgcagcgtgatgcacgaggccctgcacaaccactacacccagaagagcctgagcctgagccccggcaag

SEQ ID NO: 102 - DNA, 696 bp, synthetic construct
  source 1..696: mol_type = other DNA
gagcccaagagctgcgacaagacccacacctgccccccctgccccgcccccgagctgctgggcggccccagcgtgttcctgttcccccccaagcccaaggacaccctgatgatcagcaggacccccgaggtgacctgcgtggtggtggacgtgagccacgaggaccccgaggtgaagttcaactggtacgtggacggcgtggaggtgcacaacgccaagaccaagcccagggaggagcagtacaacagcacctacagggtggtgagcgtgctgaccgtgctgcaccaggactggctgaacggcaaggagtacaagtgcaaggtgagcaacaaggccctgcccgcccccatcgagaagaccatcagcaaggccaagggccagcccagggagccccaggtgtacaccctgccccccagcaggaaggacctgaccaagaaccaggtgagcctgacctgcctggtgaagggcttctaccccagcgacatcgccgtggagtgggagagcaacggccagcccgagaacaactacaagaccaccccccccgtgctgaagagcgacggcagcttcttcctgtacagcaagctgaccgtggacaagagcaggtggcagcagggcaacgtgttcagctgcagcgtgatgcacgaggccctgcacaaccactacacccagaagagcctgagcctgagccccggcaag

SEQ ID NO: 103 - DNA, 696 bp, synthetic construct
  source 1..696: mol_type = other DNA
gagcccaagagctgcgacaagacccacacctgccccccctgccccgcccccgagctgctgggcggccccagcgtgttcctgttcccccccaagcccaaggacaccctgatgatcagcaggacccccgaggtgacctgcgtggtggtggacgtgagccacgaggaccccgaggtgaagttcaactggtacgtggacggcgtggaggtgcacaacgccaagaccaagcccagggaggagcagtacaacagcacctacagggtggtgagcgtgctgaccgtgctgcaccaggactggctgaacggcaaggagtacaagtgcaaggtgagcaacaaggccctgcccgcccccatcgagaagaccatcagcaaggccaagggccagcccagggagcccagggtgtacaccctgccccccagcaggaaggagctgaccaagaaccaggtgagcctgacctgcctggtgaagggcttctaccccagcgacatcgccgtggagtgggagagcaacggccagcccgagaacaactacaagaccaccccccccgtgctggacagcgacggcagcttcttcctggccagcaagctgaccgtggacaagagcaggtggcagcagggcaacgtgttcagctgcagcgtgatgcacgaggccctgcacaaccactacacccagaagagcctgagcctgagccccggcaag

SEQ ID NO: 104 - DNA, 696 bp, synthetic construct
  source 1..696: mol_type = other DNA
gagcccaagagctgcgacaagacccacacctgccccccctgccccgcccccgagctgctgggcggccccagcgtgttcctgttcccccccaagcccaaggacaccctgatgatcagcaggacccccgaggtgacctgcgtggtggtggacgtgagccacgaggaccccgaggtgaagttcaactggtacgtggacggcgtggaggtgcacaacgccaagaccaagcccagggaggagcagtacaacagcacctacagggtggtgagcgtgctgaccgtgctgcaccaggactggctgaacggcaaggagtacaagtgcaaggtgagcaacaaggccctgcccgcccccatcgagaagaccatcagcaaggccaagggccagcccagggagcccagggtgtacaccctgccccccagcagggacaagctgaccaagaaccaggtgagcctgacctgcctggtgaagggcttctaccccagcgacatcgccgtggagtgggagagcaacggccagcccgagaacaactacaagaccaccccccccgtgctggacagcgacggcagcttcttcctggccagcaagctgaccgtggacaagagcaggtggcagcagggcaacgtgttcagctgcagcgtgatgcacgaggccctgcacaaccactacacccagaagagcctgagcctgagccccggcaag

SEQ ID NO: 105 - DNA, 696 bp, synthetic construct
  source 1..696: mol_type = other DNA
gagcccaagagctgcgacaagacccacacctgccccccctgccccgcccccgagctgctgggcggccccagcgtgttcctgttcccccccaagcccaaggacaccctgatgatcagcaggacccccgaggtgacctgcgtggtggtggacgtgagccacgaggaccccgaggtgaagttcaactggtacgtggacggcgtggaggtgcacaacgccaagaccaagcccagggaggagcagtacaacagcacctacagggtggtgagcgtgctgaccgtgctgcaccaggactggctgaacggcaaggagtacaagtgcaaggtgagcaacaaggccctgcccgcccccatcgagaagaccatcagcaaggccaagggccagcccagggagcccagggtgtacaccctgccccccagcagggacgagctgaccaagaaccaggtgagcctgacctgcctggtgaagggcttctaccccagcgacatcgccgtggagtgggagagcaacggccagcccgagaacaactacaagaccaccccccccgtgctgaagagcgacggcagcttcttcctgtacagcaagctgaccgtggacaagagcaggtggcagcagggcaacgtgttcagctgcagcgtgatgcacgaggccctgcacaaccactacacccagaagagcctgagcctgagccccggcaag

SEQ ID NO: 106 - DNA, 696 bp, synthetic construct
  source 1..696: mol_type = other DNA
gagcccaagagctgcgacaagacccacacctgccccccctgccccgcccccgagctgctgggcggccccagcgtgttcctgttcccccccaagcccaaggacaccctgatgatcagcaggacccccgaggtgacctgcgtggtggtggacgtgagccacgaggaccccgaggtgaagttcaactggtacgtggacggcgtggaggtgcacaacgccaagaccaagcccagggaggagcagtacaacagcacctacagggtggtgagcgtgctgaccgtgctgcaccaggactggctgaacggcaaggagtacaagtgcaaggtgagcaacaaggccctgcccgcccccatcgagaagaccatcagcaaggccaagggccagcccagggagcccagggtgtacaccctgccccccagcagggacgacctgaccaagaaccaggtgagcctgacctgcctggtgaagggcttctaccccagcgacatcgccgtggagtgggagagcaacggccagcccgagaacaactacaagaccaccccccccgtgctggacagcgacggcagcttcttcctggccagcaagctgaccgtggacaagagcaggtggcagcagggcaacgtgttcagctgcagcgtgatgcacgaggccctgcacaaccactacacccagaagagcctgagcctgagccccggcaag

SEQ ID NO: 107 - DNA, 696 bp, synthetic construct
  source 1..696: mol_type = other DNA
gagcccaagagctgcgacaagacccacacctgccccccctgccccgcccccgagctgctgggcggccccagcgtgttcctgttcccccccaagcccaaggacaccctgatgatcagcaggacccccgaggtgacctgcgtggtggtggacgtgagccacgaggaccccgaggtgaagttcaactggtacgtggacggcgtggaggtgcacaacgccaagaccaagcccagggaggagcagtacaacagcacctacagggtggtgagcgtgctgaccgtgctgcaccaggactggctgaacggcaaggagtacaagtgcaaggtgagcaacaaggccctgcccgcccccatcgagaagaccatcagcaaggccaagggccagcccagggagccccaggtgtacaccctgccccccagcagggacgagctgaccaagaaccaggtgagcctggactgcctggtgaagggcttctaccccagcgacatcgccgtggagtgggagagcaacggccagcccgagaacaactacaagaccaccccccccgtgctggacagcgacggcagcttcttcctgtacagcaagctgaccgtggacaagagcaggtggcagcagggcaacgtgttcagctgcagcgtgatgcacgaggccctgcacaaccactacacccagaagagcctgagcctgagccccggcaag

SEQ ID NO: 108 - DNA, 696 bp, synthetic construct
  source 1..696: mol_type = other DNA
gagcccaagagctgcgacaagacccacacctgccccccctgccccgcccccgagctgctgggcggccccagcgtgttcctgttcccccccaagcccaaggacaccctgatgatcagcaggacccccgaggtgacctgcgtggtggtggacgtgagccacgaggaccccgaggtgaagttcaactggtacgtggacggcgtggaggtgcacaacgccaagaccaagcccagggaggagcagtacaacagcacctacagggtggtgagcgtgctgaccgtgctgcaccaggactggctgaacggcaaggagtacaagtgcaaggtgagcaacaaggccctgcccgcccccatcgagaagaccatcagcaaggccaagggccagcccagggagccccaggtgtacaccctgccccccagcagggtggagctgaccaagaaccaggtgagcctgacctgcctggtgaagggcttctaccccagcgacatcgccgtggagtgggagagcaacggccagcccgagaacaactacaagaccaccccccccgtgctggacagcgacggcagcttcttcctgtacagcaagctgaccgtggacaagagcaggtggcagcagggcaacgtgttcagctgcagcgtgatgcacgaggccctgcacaaccactacacccagaagagcctgagcctgagccccggcaag

SEQ ID NO: 109 - DNA, 696 bp, synthetic construct
  source 1..696: mol_type = other DNA
gagcccaagagctgcgacaagacccacacctgccccccctgccccgcccccgagctgctgggcggccccagcgtgttcctgttcccccccaagcccaaggacaccctgatgatcagcaggacccccgaggtgacctgcgtggtggtggacgtgagccacgaggaccccgaggtgaagttcaactggtacgtggacggcgtggaggtgcacaacgccaagaccaagcccagggaggagcagtacaacagcacctacagggtggtgagcgtgctgaccgtgctgcaccaggactggctgaacggcaaggagtacaagtgcaaggtgagcaacaaggccctgcccgcccccatcgagaagaccatcagcaaggccaagggccagcccagggagccccaggtgtacaccctgccccccagcagggacgtgctgaccaagaaccaggtgagcctgacctgcctggtgaagggcttctaccccagcgacatcgccgtggagtgggagagcaacggccagcccgagaacaactacaagaccaccccccccgtgctggacagcgacggcagcttcttcctgtacagcaagctgaccgtggacaagagcaggtggcagcagggcaacgtgttcagctgcagcgtgatgcacgaggccctgcacaaccactacacccagaagagcctgagcctgagccccggcaag

SEQ ID NO: 110 - DNA, 696 bp, synthetic construct
  source 1..696: mol_type = other DNA
gagcccaagagctgcgacaagacccacacctgccccccctgccccgcccccgagctgctgggcggccccagcgtgttcctgttcccccccaagcccaaggacaccctgatgatcagcaggacccccgaggtgacctgcgtggtggtggacgtgagccacgaggaccccgaggtgaagttcaactggtacgtggacggcgtggaggtgcacaacgccaagaccaagcccagggaggagcagtacaacagcacctacagggtggtgagcgtgctgaccgtgctgcaccaggactggctgaacggcaaggagtacaagtgcaaggtgagcaacaaggccctgcccgcccccatcgagaagaccatcagcaaggccaagggccagcccagggagccccaggtgtacaccctgccccccagcagggacgagctgaccaagaaccaggtgagcctgacctgcctggtgaagggcttctaccccagcgacatcgccgtggagtgggagagcaacggccagcccgagaacaactacaagacctggccccccgtgctggacagcgacggcagcttcttcctgtacagcaagctgaccgtggacaagagcaggtggcagcagggcaacgtgttcagctgcagcgtgatgcacgaggccctgcacaaccactacacccagaagagcctgagcctgagccccggcaag

SEQ ID NO: 111 - DNA, 696 bp, synthetic construct
  source 1..696: mol_type = other DNA
gagcccaagagctgcgacaagacccacacctgccccccctgccccgcccccgagctgctgggcggccccagcgtgttcctgttcccccccaagcccaaggacaccctgatgatcagcaggacccccgaggtgacctgcgtggtggtggacgtgagccacgaggaccccgaggtgaagttcaactggtacgtggacggcgtggaggtgcacaacgccaagaccaagcccagggaggagcagtacaacagcacctacagggtggtgagcgtgctgaccgtgctgcaccaggactggctgaacggcaaggagtacaagtgcaaggtgagcaacaaggccctgcccgcccccatcgagaagaccatcagcaaggccaagggccagcccagggagcccatggtgtacaccctgccccccagcagggacgagctgaccaagaaccaggtgagcctgacctgcctggtgaagggcttctaccccagcgacatcgccgtggagtgggagagcaacggccagcccgagaacaactacaagaccaccccccccgtgctggacagcgacggcagcttcttcctgtacagcaagctgaccgtggacaagagcaggtggcagcagggcaacgtgttcagctgcagcgtgatgcacgaggccctgcacaaccactacacccagaagagcctgagcctgagccccggcaag

SEQ ID NO: 112 - DNA, 696 bp, synthetic construct
  source 1..696: mol_type = other DNA
gagcccaagagctgcgacaagacccacacctgccccccctgccccgcccccgagctgctgggcggccccagcgtgttcctgttcccccccaagcccaaggacaccctgatgatcagcaggacccccgaggtgacctgcgtggtggtggacgtgagccacgaggaccccgaggtgaagttcaactggtacgtggacggcgtggaggtgcacaacgccaagaccaagcccagggaggagcagtacaacagcacctacagggtggtgagcgtgctgaccgtgctgcaccaggactggctgaacggcaaggagtacaagtgcaaggtgagcaacaaggccctgcccgcccccatcgagaagaccatcagcaaggccaagggccagcccagggagccccaggtgtacaccctgccccccagcagggacgagctgaccaagaaccaggtgagcctgagctgcgccgtgaagggcttctaccccagcgacatcgccgtggagtgggagagcaacggccagcccgagaacaactacaagaccaccccccccgtgctggacagcgacggcagcttcttcctggtgagctggctgaccgtggacaagagcaggtggcagcagggcaacgtgttcagctgcagcgtgatgcacgaggccctgcacaaccactacacccagaagagcctgagcctgagccccggcaag

SEQ ID NO: 113 - DNA, 696 bp, synthetic construct
  source 1..696: mol_type = other DNA
gagcccaagagctgcgacaagacccacacctgccccccctgccccgcccccgagctgctgggcggccccagcgtgttcctgttcccccccaagcccaaggacaccctgatgatcagcaggacccccgaggtgacctgcgtggtggtggacgtgagccacgaggaccccgaggtgaagttcaactggtacgtggacggcgtggaggtgcacaacgccaagaccaagcccagggaggagcagtacaacagcacctacagggtggtgagcgtgctgaccgtgctgcaccaggactggctgaacggcaaggagtacaagtgcaaggtgagcaacaaggccctgcccgcccccatcgagaagaccatcagcaaggccaagggccagcccagggagccccaggtgtacaccctgccccccagcagggacgagctgaccaagaaccaggtgagcctgagctgcgccgtggagggcttctaccccagcgacatcgccgtggagtgggagagcaacggccagcccgagaacaactacaagaccaccccccccgtgctggacagcgacggcagcttcttcctggtgagcgacctgaccgtggacaagagcaggtggcagcagggcaacgtgttcagctgcagcgtgatgcacgaggccctgcacaaccactacacccagaagagcctgagcctgagccccggcaag

SEQ ID NO: 114 - DNA, 696 bp, synthetic construct
  source 1..696: mol_type = other DNA
gagcccaagagctgcgacaagacccacacctgccccccctgccccgcccccgagctgctgggcggccccagcgtgttcctgttcccccccaagcccaaggacaccctgatgatcagcaggacccccgaggtgacctgcgtggtggtggacgtgagccacgaggaccccgaggtgaagttcaactggtacgtggacggcgtggaggtgcacaacgccaagaccaagcccagggaggagcagtacaacagcacctacagggtggtgagcgtgctgaccgtgctgcaccaggactggctgaacggcaaggagtacaagtgcaaggtgagcaacaaggccctgcccgcccccatcgagaagaccatcagcaaggccaagggccagcccagggagccccaggtgtacaccctgccccccagcagggacgagctgaccaagaaccaggtgagcctgacctgcctggtgaagggcttctaccccagcgacatcgccgtggagtgggagagcaacggccagcccgagaacaactacaagaccaccccccccgtgctggacagcgacggcagcttcttcctggccagctggctgaccgtggacaagagcaggtggcagcagggcaacgtgttcagctgcagcgtgatgcacgaggccctgcacaaccactacacccagaagagcctgagcctgagccccggcaag

SEQ ID NO: 115 - DNA, 696 bp, synthetic construct
  source 1..696: mol_type = other DNA
gagcccaagagctgcgacaagacccacacctgccccccctgccccgcccccgagctgctgggcggccccagcgtgttcctgttcccccccaagcccaaggacaccctgatgatcagcaggacccccgaggtgacctgcgtggtggtggacgtgagccacgaggaccccgaggtgaagttcaactggtacgtggacggcgtggaggtgcacaacgccaagaccaagcccagggaggagcagtacaacagcacctacagggtggtgagcgtgctgaccgtgctgcaccaggactggctgaacggcaaggagtacaagtgcaaggtgagcaacaaggccctgcccgcccccatcgagaagaccatcagcaaggccaagggccagcccagggagccccaggtgtacaccctgccccccagcagggacgagctgaccaagaaccaggtgagcctgacctgcctggtggagggcttctaccccagcgacatcgccgtggagtgggagagcaacggccagcccgagaacaactacaagaccaccccccccgtgctggacagcgacggcagcttcttcctggccagcgacctgaccgtggacaagagcaggtggcagcagggcaacgtgttcagctgcagcgtgatgcacgaggccctgcacaaccactacacccagaagagcctgagcctgagccccggcaag

SEQ ID NO: 116 - DNA, 696 bp, synthetic construct
  source 1..696: mol_type = other DNA
gagcccaagagctgcgacaagacccacacctgccccccctgccccgcccccgagctgctgggcggccccagcgtgttcctgttcccccccaagcccaaggacaccctgatgatcagcaggacccccgaggtgacctgcgtggtggtggacgtgagccacgaggaccccgaggtgaagttcaactggtacgtggacggcgtggaggtgcacaacgccaagaccaagcccagggaggagcagtacaacagcacctacagggtggtgagcgtgctgaccgtgctgcaccaggactggctgaacggcaaggagtacaagtgcaaggtgagcaacaaggccctgcccgcccccatcgagaagaccatcagcaaggccaagggccagcccagggagccccaggtgtacaccctgccccccagcagggacgagctgaccaagaaccaggtgagcctgagctgcgccgtgaagggcttctaccccagcgacatcgccgtggagtgggagagcaacggccagcccgagaacaactacaagaccaccccccccgtgctggacagcgacggcagcttcttcctggtgagcaagctgaccgtggacaagagcaggtggcagcagggcaacgtgttcagctgcagcgtgatgcacgaggccctgcacaaccactacacccaggagagcctgagcctgagccccggcaag

SEQ ID NO: 117 - DNA, 696 bp, synthetic construct
  source 1..696: mol_type = other DNA
gagcccaagagctgcgacaagacccacacctgccccccctgccccgcccccgagctgctgggcggccccagcgtgttcctgttcccccccaagcccaaggacaccctgatgatcagcaggacccccgaggtgacctgcgtggtggtggacgtgagccacgaggaccccgaggtgaagttcaactggtacgtggacggcgtggaggtgcacaacgccaagaccaagcccagggaggagcagtacaacagcacctacagggtggtgagcgtgctgaccgtgctgcaccaggactggctgaacggcaaggagtacaagtgcaaggtgagcaacaaggccctgcccgcccccatcgagaagaccatcagcaaggccaagggccagcccagggagccccaggtgtacaccctgccccccagcagggacgagctgaccaagaaccaggtgagcctgagctgcgccgtgtacggcttctaccccagcgacatcgccgtggagtgggagagcaacggccagcccgagaacaactacaagaccaccccccccgtgctggacagcgacggcagcttcttcctggtgagcaagctgaccgtggacaagagcaggtggcagcagggcaacgtgttcagctgcagcgtgatgcacgaggccctgcacaaccactacacccagaagagcctgagcctgagccccggcaag

SEQ ID NO: 118 - DNA, 696 bp, synthetic construct
  source 1..696: mol_type = other DNA
gagcccaagagctgcgacaagacccacacctgccccccctgccccgcccccgagctgctgggcggccccagcgtgttcctgttcccccccaagcccaaggacaccctgatgatcagcaggacccccgaggtgacctgcgtggtggtggacgtgagccacgaggaccccgaggtgaagttcaactggtacgtggacggcgtggaggtgcacaacgccaagaccaagcccagggaggagcagtacaacagcacctacagggtggtgagcgtgctgaccgtgctgcaccaggactggctgaacggcaaggagtacaagtgcaaggtgagcaacaaggccctgcccgcccccatcgagaagaccatcagcaaggccaagggccagcccagggagccccaggtgtacaccctgccccccagcagggacgagctgaccgacaaccaggtgagcctgagctgcgccgtgaagggcttctaccccagcgacatcgccgtggagtgggagagcaacggccagcccgagaacaactacaagaccaccccccccgtgctggacagcgacggcagcttcttcctggtgagcaagctgaccgtggacaagagcaggtggcagcagggcaacgtgttcagctgcagcgtgatgcacgaggccctgcacaaccactacacccagaagagcctgagcctgagccccggcaag

SEQ ID NO: 119 - DNA, 696 bp, synthetic construct
  source 1..696: mol_type = other DNA
gagcccaagagctgcgacaagacccacacctgccccccctgccccgcccccgagctgctgggcggccccagcgtgttcctgttcccccccaagcccaaggacaccctgatgatcagcaggacccccgaggtgacctgcgtggtggtggacgtgagccacgaggaccccgaggtgaagttcaactggtacgtggacggcgtggaggtgcacaacgccaagaccaagcccagggaggagcagtacaacagcacctacagggtggtgagcgtgctgaccgtgctgcaccaggactggctgaacggcaaggagtacaagtgcaaggtgagcaacaaggccctgcccgcccccatcgagaagaccatcagcaaggccaagggccagcccagggagccccaggtgtacaccctgccccccagcagggacgagctgaccaagaaccaggtgagcctgacctgcctggtgaagggcttctaccccagcgacatcgccgtggagtgggagagcaacggccagcccgagaacaactacaagaccaccccccccgtgctggacagcgacggcagcttcttcctggccagcaagctgaccgtggacaagagcaggtggcagcagggcaacgtgttcagctgcagcgtgatgcacgaggccctgcacaaccactacacccaggagagcctgagcctgagccccggcaag

SEQ ID NO: 120 - DNA, 696 bp, synthetic construct; identical to SEQ ID NO: 93
  source 1..696: mol_type = other DNA

SEQ ID NO: 121 - DNA, 696 bp, synthetic construct
  source 1..696: mol_type = other DNA
gagcccaagagctgcgacaagacccacacctgccccccctgccccgcccccgagctgctgggcggccccagcgtgttcctgttcccccccaagcccaaggacaccctgatgatcagcaggacccccgaggtgacctgcgtggtggtggacgtgagccacgaggaccccgaggtgaagttcaactggtacgtggacggcgtggaggtgcacaacgccaagaccaagcccagggaggagcagtacaacagcacctacagggtggtgagcgtgctgaccgtgctgcaccaggactggctgaacggcaaggagtacaagtgcaaggtgagcaacaaggccctgcccgcccccatcgagaagaccatcagcaaggccaagggccagcccagggagccccaggtgtacaccctgccccccagcagggacgagctgaccgacaaccaggtgagcctgacctgcctggtgaagggcttctaccccagcgacatcgccgtggagtgggagagcaacggccagcccgagaacaactacaagaccaccccccccgtgctggacagcgacggcagcttcttcctggccagcaagctgaccgtggacaagagcaggtggcagcagggcaacgtgttcagctgcagcgtgatgcacgaggccctgcacaaccactacacccagaagagcctgagcctgagccccggcaag

SEQ ID NO: 122 - DNA, 696 bp, synthetic construct
  source 1..696: mol_type = other DNA
gagcccaagagctgcgacaagacccacacctgccccccctgccccgcccccgagctgctgggcggccccagcgtgttcctgttcccccccaagcccaaggacaccctgatgatcagcaggacccccgaggtgacctgcgtggtggtggacgtgagccacgaggaccccgaggtgaagttcaactggtacgtggacggcgtggaggtgcacaacgccaagaccaagcccagggaggagcagtacaacagcacctacagggtggtgagcgtgctgaccgtgctgcaccaggactggctgaacggcaaggagtacaagtgcaaggtgagcaacaaggccctgcccgcccccatcgagaagaccatcagcaaggccaagggccagcccagggagccccaggtgtacaccctgccccccagcagggacgagctgaccaagaaccaggtgagcctgagctgcgccgtgaagggcttctaccccagcgacatcgccgtggagtgggagagcaacggccagcccgagaacaactacaagaccaccccccccgtgctggtgagcgacggcagcttcaccctggtgagcaagctgaccgtggacaagagcaggtggcagcagggcaacgtgttcagctgcagcgtgatgcacgaggccctgcacaaccactacacccagaagagcctgagcctgagccccggcaag

SEQ ID NO: 123 - DNA, 696 bp, synthetic construct
  source 1..696: mol_type = other DNA
gagcccaagagctgcgacaagacccacacctgccccccctgccccgcccccgagctgctgggcggccccagcgtgttcctgttcccccccaagcccaaggacaccctgatgatcagcaggacccccgaggtgacctgcgtggtggtggacgtgagccacgaggaccccgaggtgaagttcaactggtacgtggacggcgtggaggtgcacaacgccaagaccaagcccagggaggagcagtacaacagcacctacagggtggtgagcgtgctgaccgtgctgcaccaggactggctgaacggcaaggagtacaagtgcaaggtgagcaacaaggccctgcccgcccccatcgagaagaccatcagcaaggccaagggccagcccagggagccccaggtgtacaccctgccccccagcagggacaagctgaccaagaaccaggtgagcctgagctgcgccgtgaagggcttctaccccagcgacatcgccgtggagtgggagagcaacggccagcccgagaacaactacaagaccaccccccccgtgctgaagagcgacggcagcttcttcctggtgagcaagctgaccgtggacaagagcaggtggcagcagggcaacgtgttcagctgcagcgtgatgcacgaggccctgcacaaccactacacccagaagagcctgagcctgagccccggcaag

SEQ ID NO: 124 - DNA, 696 bp, synthetic construct
  source 1..696: mol_type = other DNA
gagcccaagagctgcgacaagacccacacctgccccccctgccccgcccccgagctgctgggcggccccagcgtgttcctgttcccccccaagcccaaggacaccctgatgatcagcaggacccccgaggtgacctgcgtggtggtggacgtgagccacgaggaccccgaggtgaagttcaactggtacgtggacggcgtggaggtgcacaacgccaagaccaagcccagggaggagcagtacaacagcacctacagggtggtgagcgtgctgaccgtgctgcaccaggactggctgaacggcaaggagtacaagtgcaaggtgagcaacaaggccctgcccgcccccatcgagaagaccatcagcaaggccaagggccagcccagggagccccaggtgtacaccctgccccccagcagggacgagctgaccaagaaccaggtgagcctgacctgcctggtgaagggcttctaccccagcgacatcgccgtggagtgggagagcaacggccagcccgagaacaactacaagaccaccccccccgtgctggtgagcgacggcagcttcaccctggccagcaagctgaccgtggacaagagcaggtggcagcagggcaacgtgttcagctgcagcgtgatgcacgaggccctgcacaaccactacacccagaagagcctgagcctgagccccggcaag

SEQ ID NO: 125 - DNA, 696 bp, synthetic construct
  source 1..696: mol_type = other DNA
gagcccaagagctgcgacaagacccacacctgccccccctgccccgcccccgagctgctgggcggccccagcgtgttcctgttcccccccaagcccaaggacaccctgatgatcagcaggacccccgaggtgacctgcgtggtggtggacgtgagccacgaggaccccgaggtgaagttcaactggtacgtggacggcgtggaggtgcacaacgccaagaccaagcccagggaggagcagtacaacagcacctacagggtggtgagcgtgctgaccgtgctgcaccaggactggctgaacggcaaggagtacaagtgcaaggtgagcaacaaggccctgcccgcccccatcgagaagaccatcagcaaggccaagggccagcccagggagccccaggtgtacaccctgccccccagcagggacaagctgaccaagaaccaggtgagcctgacctgcctggtgaagggcttctaccccagcgacatcgccgtggagtgggagagcaacggccagcccgagaacaactacaagaccaccccccccgtgctgaagagcgacggcagcttcttcctggccagcaagctgaccgtggacaagagcaggtggcagcagggcaacgtgttcagctgcagcgtgatgcacgaggccctgcacaaccactacacccagaagagcctgagcctgagccccggcaag

SEQ ID NO: 126 - DNA, 696 bp, synthetic construct
  source 1..696: mol_type = other DNA
gagcccaagagctgcgacaagacccacacctgccccccctgccccgcccccgagctgctgggcggccccagcgtgttcctgttcccccccaagcccaaggacaccctgatgatcagcaggacccccgaggtgacctgcgtggtggtggacgtgagccacgaggaccccgaggtgaagttcaactggtacgtggacggcgtggaggtgcacaacgccaagaccaagcccagggaggagcagtacaacagcacctacagggtggtgagcgtgctgaccgtgctgcaccaggactggctgaacggcaaggagtacaagtgcaaggtgagcaacaaggccctgcccgcccccatcgagaagaccatcagcaaggccaagggccagcccagggagccccaggtgtacaccctgccccccagcaggaaggagctgaccaagaaccaggtgagcctgagctgcgccgtgaagggcttctaccccagcgacatcgccgtggagtgggagagcaacggccagcccgagaacaactacaagaccaccccccccgtgctggacagcgacggcagcttcttcctggtgagcaagctgaccgtggacaagagcaggtggcagcagggcaacgtgttcagctgcagcgtgatgcacgaggccctgcacaaccactacacccagaagagcctgagcctgagccccggcaag

SEQ ID NO: 127 - DNA, 696 bp, synthetic construct
  source 1..696: mol_type = other DNA
gagcccaagagctgcgacaagacccacacctgccccccctgccccgcccccgagctgctgggcggccccagcgtgttcctgttcccccccaagcccaaggacaccctgatgatcagcaggacccccgaggtgacctgcgtggtggtggacgtgagccacgaggaccccgaggtgaagttcaactggtacgtggacggcgtggaggtgcacaacgccaagaccaagcccagggaggagcagtacaacagcacctacagggtggtgagcgtgctgaccgtgctgcaccaggactggctgaacggcaaggagtacaagtgcaaggtgagcaacaaggccctgcccgcccccatcgagaagaccatcagcaaggccaagggccagcccagggagccccaggtgtacaccctgccccccagcagggacgacctgaccaagaaccaggtgagcctgagctgcgccgtgaagggcttctaccccagcgacatcgccgtggagtgggagagcaacggccagcccgagaacaactacaagaccaccccccccgtgctggacagcgacggcagcttcttcctggtgagcaagctgaccgtggacaagagcaggtggcagcagggcaacgtgttcagctgcagcgtgatgcacgaggccctgcacaaccactacacccagaagagcctgagcctgagccccggcaag

SEQ ID NO: 128 - DNA, 696 bp, synthetic construct
  source 1..696: mol_type = other DNA
gagcccaagagctgcgacaagacccacacctgccccccctgccccgcccccgagctgctgggcggccccagcgtgttcctgttcccccccaagcccaaggacaccctgatgatcagcaggacccccgaggtgacctgcgtggtggtggacgtgagccacgaggaccccgaggtgaagttcaactggtacgtggacggcgtggaggtgcacaacgccaagaccaagcccagggaggagcagtacaacagcacctacagggtggtgagcgtgctgaccgtgctgcaccaggactggctgaacggcaaggagtacaagtgcaaggtgagcaacaaggccctgcccgcccccatcgagaagaccatcagcaaggccaagggccagcccagggagcccagggtgtacaccctgccccccagcagggacgagctgaccaagaaccaggtgagcctgagctgcgccgtgaagggcttctaccccagcgacatcgccgtggagtgggagagcaacggccagcccgagaacaactacaagaccaccccccccgtgctggacagcgacggcagcttcttcctggtgagcaagctgaccgtggacaagagcaggtggcagcagggcaacgtgttcagctgcagcgtgatgcacgaggccctgcacaaccactacacccagaagagcctgagcctgagccccggcaag

SEQ ID NO: 129 - DNA, 696 bp, synthetic construct
  source 1..696: mol_type = other DNA
gagcccaagagctgcgacaagacccacacctgccccccctgccccgcccccgagctgctgggcggccccagcgtgttcctgttcccccccaagcccaaggacaccctgatgatcagcaggacccccgaggtgacctgcgtggtggtggacgtgagccacgaggaccccgaggtgaagttcaactggtacgtggacggcgtggaggtgcacaacgccaagaccaagcccagggaggagcagtacaacagcacctacagggtggtgagcgtgctgaccgtgctgcaccaggactggctgaacggcaaggagtacaagtgcaaggtgagcaacaaggccctgcccgcccccatcgagaagaccatcagcaaggccaagggccagcccagggagccccaggtgtacaccctgccccccagcaggaaggagctgaccaagaaccaggtgagcctgacctgcctggtgaagggcttctaccccagcgacatcgccgtggagtgggagagcaacggccagcccgagaacaactacaagaccaccccccccgtgctggacagcgacggcagcttcttcctggccagcaagctgaccgtggacaagagcaggtggcagcagggcaacgtgttcagctgcagcgtgatgcacgaggccctgcacaaccactacacccagaagagcctgagcctgagccccggcaag

SEQ ID NO: 130 - DNA, 696 bp, synthetic construct; identical to SEQ ID NO: 83
  source 1..696: mol_type = other DNA

SEQ ID NO: 131 - DNA, 696 bp, synthetic construct
  source 1..696: mol_type = other DNA
gagcccaagagctgcgacaagacccacacctgccccccctgccccgcccccgagctgctgggcggccccagcgtgttcctgttcccccccaagcccaaggacaccctgatgatcagcaggacccccgaggtgacctgcgtggtggtggacgtgagccacgaggaccccgaggtgaagttcaactggtacgtggacggcgtggaggtgcacaacgccaagaccaagcccagggaggagcagtacaacagcacctacagggtggtgagcgtgctgaccgtgctgcaccaggactggctgaacggcaaggagtacaagtgcaaggtgagcaacaaggccctgcccgcccccatcgagaagaccatcagcaaggccaagggccagcccagggagcccagggtgtacaccctgccccccagcagggacgagctgaccaagaaccaggtgagcctgacctgcctggtgaagggcttctaccccagcgacatcgccgtggagtgggagagcaacggccagcccgagaacaactacaagaccaccccccccgtgctggacagcgacggcagcttcttcctggccagcaagctgaccgtggacaagagcaggtggcagcagggcaacgtgttcagctgcagcgtgatgcacgaggccctgcacaaccactacacccagaagagcctgagcctgagccccggcaag

SEQ ID NO: 132 - DNA, 696 bp, synthetic construct
  source 1..696: mol_type = other DNA
gagcccaagagctgcgacaagacccacacctgccccccctgccccgcccccgagctgctgggcggccccagcgtgttcctgttcccccccaagcccaaggacaccctgatgatcagcaggacccccgaggtgacctgcgtggtggtggacgtgagccacgaggaccccgaggtgaagttcaactggtacgtggacggcgtggaggtgcacaacgccaagaccaagcccagggaggagcagtacaacagcacctacagggtggtgagcgtgctgaccgtgctgcaccaggactggctgaacggcaaggagtacaagtgcaaggtgagcaacaaggccctgcccgcccccatcgagaagaccatcagcaaggccaagggccagcccagggagccccaggtgtacaccctgccccccagcagggacgagctgaccaagaaccaggtgagcctgacctgcctggtgaagggcttctaccccagcgacatcgccgtggagtgggagagcaacggccagcccgagaacaactacaagaccaccccccccgtgctggacagcgacggcagcttcttcctgtacagctggctgaccgtggacaagagcaggtggcagcagggcaacgtgttcagctgcagcgtgatgcacgaggccctgcacaaccactacacccaggagagcctgagcctgagccccggcaag

SEQ ID NO: 133 - DNA, 696 bp, synthetic construct
  source 1..696: mol_type = other DNA
gagcccaagagctgcgacaagacccacacctgccccccctgccccgcccccgagctgctgggcggccccagcgtgttcctgttcccccccaagcccaaggacaccctgatgatcagcaggacccccgaggtgacctgcgtggtggtggacgtgagccacgaggaccccgaggtgaagttcaactggtacgtggacggcgtggaggtgcacaacgccaagaccaagcccagggaggagcagtacaacagcacctacagggtggtgagcgtgctgaccgtgctgcaccaggactggctgaacggcaaggagtacaagtgcaaggtgagcaacaaggccctgcccgcccccatcgagaagaccatcagcaaggccaagggccagcccagggagccccaggtgtacaccctgccccccagcagggacgagctgaccaagaaccaggtgagcctgacctgcctggtggagggcttctaccccagcgacatcgccgtggagtgggagagcaacggccagcccgagaacaactacaagaccaccccccccgtgctggacagcgacggcagcttcttcctgtacagctggctgaccgtggacaagagcaggtggcagcagggcaacgtgttcagctgcagcgtgatgcacgaggccctgcacaaccactacacccagaagagcctgagcctgagccccggcaag

SEQ ID NO: 134 - DNA, 696 bp, synthetic construct
  source 1..696: mol_type = other DNA
gagcccaagagctgcgacaagacccacacctgccccccctgccccgcccccgagctgctgggcggccccagcgtgttcctgttcccccccaagcccaaggacaccctgatgatcagcaggacccccgaggtgacctgcgtggtggtggacgtgagccacgaggaccccgaggtgaagttcaactggtacgtggacggcgtggaggtgcacaacgccaagaccaagcccagggaggagcagtacaacagcacctacagggtggtgagcgtgctgaccgtgctgcaccaggactggctgaacggcaaggagtacaagtgcaaggtgagcaacaaggccctgcccgcccccatcgagaagaccatcagcaaggccaagggccagcccagggagccccaggtgtacaccctgccccccagcagggacgagctgaccaagaaccaggtgagcctgacctgcctggtgtacggcttctaccccagcgacatcgccgtggagtgggagagcaacggccagcccgagaacaactacaagaccaccccccccgtgctggacagcgacggcagcttcttcctgtacagctggctgaccgtggacaagagcaggtggcagcagggcaacgtgttcagctgcagcgtgatgcacgaggccctgcacaaccactacacccagaagagcctgagcctgagccccggcaag

SEQ ID NO: 135 - DNA, 696 bp, synthetic construct
  source 1..696: mol_type = other DNA
gagcccaagagctgcgacaagacccacacctgccccccctgccccgcccccgagctgctgggcggccccagcgtgttcctgttcccccccaagcccaaggacaccctgatgatcagcaggacccccgaggtgacctgcgtggtggtggacgtgagccacgaggaccccgaggtgaagttcaactggtacgtggacggcgtggaggtgcacaacgccaagaccaagcccagggaggagcagtacaacagcacctacagggtggtgagcgtgctgaccgtgctgcaccaggactggctgaacggcaaggagtacaagtgcaaggtgagcaacaaggccctgcccgcccccatcgagaagaccatcagcaaggccaagggccagcccagggagccccaggtgtacaccctgccccccagcagggacgagctgaccaagaaccaggtgagcctgacctgcctggtgtacggcttctaccccagcgacatcgccgtggagtgggagagcaacggccagcccgagaacaactacaagaccaccccccccgtgctggacagcgacggcagcttcttcctgtacagcgtgctgaccgtggacaagagcaggtggcagcagggcaacgtgttcagctgcagcgtgatgcacgaggccctgcacaaccactacacccaggagagcctgagcctgagccccggcaag

SEQ ID NO: 136 - DNA, 696 bp, synthetic construct
  source 1..696: mol_type = other DNA
gagcccaagagctgcgacaagacccacacctgccccccctgccccgcccccgagctgctgggcggccccagcgtgttcctgttcccccccaagcccaaggacaccctgatgatcagcaggacccccgaggtgacctgcgtggtggtggacgtgagccacgaggaccccgaggtgaagttcaactggtacgtggacggcgtggaggtgcacaacgccaagaccaagcccagggaggagcagtacaacagcacctacagggtggtgagcgtgctgaccgtgctgcaccaggactggctgaacggcaaggagtacaagtgcaaggtgagcaacaaggccctgcccgcccccatcgagaagaccatcagcaaggccaagggccagcccagggagccccaggtgtacaccctgccccccagcagggacgagctgaccaagaaccaggtgagcctgacctgcctggtgtacggcttctaccccagcgacatcgccgtggagtgggagagcaacggccagcccgagaacaactacaagaccaccccccccgtgctggacagcgacggcagcttcttcctgtacagcgacctgaccgtggacaagagcaggtggcagcagggcaacgtgttcagctgcagcgtgatgcacgaggccctgcacaaccactacacccagaagagcctgagcctgagccccggcaag

SEQ ID NO: 137 - DNA, 696 bp, synthetic construct
  source 1..696: mol_type = other DNA
gagcccaagagctgcgacaagacccacacctgccccccctgccccgcccccgagctgctgggcggccccagcgtgttcctgttcccccccaagcccaaggacaccctgatgatcagcaggacccccgaggtgacctgcgtggtggtggacgtgagccacgaggaccccgaggtgaagttcaactggtacgtggacggcgtggaggtgcacaacgccaagaccaagcccagggaggagcagtacaacagcacctacagggtggtgagcgtgctgaccgtgctgcaccaggactggctgaacggcaaggagtacaagtgcaaggtgagcaacaaggccctgcccgcccccatcgagaagaccatcagcaaggccaagggccagcccagggagccccaggtgtacaccctgccccccagcagggacgagctgaccaagaaccaggtgagcctgacctgcctggtggagggcttctaccccagcgacatcgccgtggagtgggagagcaacggccagcccgagaacaactacaagaccaccccccccgtgctggacagcgacggcagcttcttcctgtacagctggctgaccgtggacaagagcaggtggcagcagggcaacgtgttcagctgcagcgtgatgcacgaggccctgcacaaccactacacccaggagagcctgagcctgagccccggcaag

SEQ ID NO: 138 - DNA, 696 bp, synthetic construct
  source 1..696: mol_type = other DNA
gagcccaagagctgcgacaagacccacacctgccccccctgccccgcccccgagctgctgggcggccccagcgtgttcctgttcccccccaagcccaaggacaccctgatgatcagcaggacccccgaggtgacctgcgtggtggtggacgtgagccacgaggaccccgaggtgaagttcaactggtacgtggacggcgtggaggtgcacaacgccaagaccaagcccagggaggagcagtacaacagcacctacagggtggtgagcgtgctgaccgtgctgcaccaggactggctgaacggcaaggagtacaagtgcaaggtgagcaacaaggccctgcccgcccccatcgagaagaccatcagcaaggccaagggccagcccagggagccccaggtgtacaccctgccccccagcagggacgagctgaccaagaaccaggtgagcctgacctgcctggtgtacggcttctaccccagcgacatcgccgtggagtgggagagcaacggccagcccgagaacaactacaagaccaccccccccgtgctggacagcgacggcagcttcttcctgtacagctggctgaccgtggacaagagcaggtggcagcagggcaacgtgttcagctgcagcgtgatgcacgaggccctgcacaaccactacacccaggagagcctgagcctgagccccggcaag

SEQ ID NO: 139 - DNA, 696 bp, synthetic construct
  source 1..696: mol_type = other DNA
gagcccaagagctgcgacaagacccacacctgccccccctgccccgcccccgagctgctgggcggccccagcgtgttcctgttcccccccaagcccaaggacaccctgatgatcagcaggacccccgaggtgacctgcgtggtggtggacgtgagccacgaggaccccgaggtgaagttcaactggtacgtggacggcgtggaggtgcacaacgccaagaccaagcccagggaggagcagtacaacagcacctacagggtggtgagcgtgctgaccgtgctgcaccaggactggctgaacggcaaggagtacaagtgcaaggtgagcaacaaggccctgcccgcccccatcgagaagaccatcagcaaggccaagggccagcccagggagccccaggtgtacaccctgccccccagcagggacgagctgaccaagaaccaggtgagcctgacctgcctggtgtacggcttctaccccagcgacatcgccgtggagtgggagagcaacggccagcccgagaacaactacaagaccaccccccccgtgctggacagcgacggcagcttcttcctgtacagcgacctgaccgtggacaagagcaggtggcagcagggcaacgtgttcagctgcagcgtgatgcacgaggccctgcacaaccactacacccaggagagcctgagcctgagccccggcaag

SEQ ID NO: 140 - DNA, 696 bp, synthetic construct
  source 1..696: mol_type = other DNA
gagcccaagagctgcgacaagacccacacctgccccccctgccccgcccccgagctgctgggcggccccagcgtgttcctgttcccccccaagcccaaggacaccctgatgatcagcaggacccccgaggtgacctgcgtggtggtggacgtgagccacgaggaccccgaggtgaagttcaactggtacgtggacggcgtggaggtgcacaacgccaagaccaagcccagggaggagcagtacaacagcacctacagggtggtgagcgtgctgaccgtgctgcaccaggactggctgaacggcaaggagtacaagtgcaaggtgagcaacaaggccctgcccgcccccatcgagaagaccatcagcaaggccaagggccagcccagggagccccaggtgtacaccctgccccccagcagggacgagctgaccgacaaccaggtgagcctgacctgcctggtgaagggcttctaccccagcgacatcgccgtggagtgggagagcaacggccagcccgagaacaactacaagaccaccccccccgtgctggacagcgacggcagcttcttcctgtacagcgtgctgaccgtggacaagagcaggtggcagcagggcaacgtgttcagctgcagcgtgatgcacgaggccctgcacaaccactacacccaggagagcctgagcctgagccccggcaag

SEQ ID NO: 141 - DNA, 696 bp, synthetic construct
  source 1..696: mol_type = other DNA
gagcccaagagctgcgacaagacccacacctgccccccctgccccgcccccgagctgctgggcggccccagcgtgttcctgttcccccccaagcccaaggacaccctgatgatcagcaggacccccgaggtgacctgcgtggtggtggacgtgagccacgaggaccccgaggtgaagttcaactggtacgtggacggcgtggaggtgcacaacgccaagaccaagcccagggaggagcagtacaacagcacctacagggtggtgagcgtgctgaccgtgctgcaccaggactggctgaacggcaaggagtacaagtgcaaggtgagcaacaaggccctgcccgcccccatcgagaagaccatcagcaaggccaagggccagcccagggagccccaggtgtacaccctgccccccagcagggacgagctgaccgacaaccaggtgagcctgacctgcctggtggagggcttctaccccagcgacatcgccgtggagtgggagagcaacggccagcccgagaacaactacaagaccaccccccccgtgctggacagcgacggcagcttcttcctgtacagcgtgctgaccgtggacaagagcaggtggcagcagggcaacgtgttcagctgcagcgtgatgcacgaggccctgcacaaccactacacccagaagagcctgagcctgagccccggcaag

SEQ ID NO: 142 - DNA, 696 bp, synthetic construct
  source 1..696: mol_type = other DNA
gagcccaagagctgcgacaagacccacacctgccccccctgccccgcccccgagctgctgggcggccccagcgtgttcctgttcccccccaagcccaaggacaccctgatgatcagcaggacccccgaggtgacctgcgtggtggtggacgtgagccacgaggaccccgaggtgaagttcaactggtacgtggacggcgtggaggtgcacaacgccaagaccaagcccagggaggagcagtacaacagcacctacagggtggtgagcgtgctgaccgtgctgcaccaggactggctgaacggcaaggagtacaagtgcaaggtgagcaacaaggccctgcccgcccccatcgagaagaccatcagcaaggccaagggccagcccagggagccccaggtgtacaccctgccccccagcagggacgagctgaccgacaaccaggtgagcctgacctgcctggtgaagggcttctaccccagcgacatcgccgtggagtgggagagcaacggccagcccgagaacaactacaagaccaccccccccgtgctggacagcgacggcagcttcttcctgtacagcgacctgaccgtggacaagagcaggtggcagcagggcaacgtgttcagctgcagcgtgatgcacgaggccctgcacaaccactacacccagaagagcctgagcctgagccccggcaag

SEQ ID NO: 143 - DNA, 696 bp, synthetic construct
  source 1..696: mol_type = other DNA
gagcccaagagctgcgacaagacccacacctgccccccctgccccgcccccgagctgctgggcggccccagcgtgttcctgttcccccccaagcccaaggacaccctgatgatcagcaggacccccgaggtgacctgcgtggtggtggacgtgagccacgaggaccccgaggtgaagttcaactggtacgtggacggcgtggaggtgcacaacgccaagaccaagcccagggaggagcagtacaacagcacctacagggtggtgagcgtgctgaccgtgctgcaccaggactggctgaacggcaaggagtacaagtgcaaggtgagcaacaaggccctgcccgcccccatcgagaagaccatcagcaaggccaagggccagcccagggagccccaggtgtacaccctgccccccagcagggacgagctgaccgacaaccaggtgagcctgacctgcctggtgtacggcttctaccccagcgacatcgccgtggagtgggagagcaacggccagcccgagaacaactacaagaccaccccccccgtgctggacagcgacggcagcttcttcctgtacagcgtgctgaccgtggacaagagcaggtggcagcagggcaacgtgttcagctgcagcgtgatgcacgaggccctgcacaaccactacacccagaagagcctgagcctgagccccggcaag

SEQ ID NO: 144 - DNA, 696 bp, synthetic construct
  source 1..696: mol_type = other DNA
gagcccaagagctgcgacaagacccacacctgccccccctgccccgcccccgagctgctgggcggccccagcgtgttcctgttcccccccaagcccaaggacaccctgatgatcagcaggacccccgaggtgacctgcgtggtggtggacgtgagccacgaggaccccgaggtgaagttcaactggtacgtggacggcgtggaggtgcacaacgccaagaccaagcccagggaggagcagtacaacagcacctacagggtggtgagcgtgctgaccgtgctgcaccaggactggctgaacggcaaggagtacaagtgcaaggtgagcaacaaggccctgcccgcccccatcgagaagaccatcagcaaggccaagggccagcccagggagccccaggtgtacaccctgccccccagcagggacgagctgaccaagaaccaggtgagcctgacctgcctggtgaagggcttctaccccagcgacatcgccgtggagtgggagagcaacggccagcccgagaacaactacaagaccaccccccccgtgctggacagcgacggcagcttcttcctgaagagcaagctgaccgtggacaagagcaggtggcagcagggcaacgtgttcagctgcagcgtgatgcacgaggccctgcacaaccactacacccagaagagcctgagcctgagccccggcaag

SEQ ID NO: 145 - DNA, 696 bp, synthetic construct
  source 1..696: mol_type = other DNA
gagcccaagagctgcgacaagacccacacctgccccccctgccccgcccccgagctgctgggcggccccagcgtgttcctgttcccccccaagcccaaggacaccctgatgatcagcaggacccccgaggtgacctgcgtggtggtggacgtgagccacgaggaccccgaggtgaagttcaactggtacgtggacggcgtggaggtgcacaacgccaagaccaagcccagggaggagcagtacaacagcacctacagggtggtgagcgtgctgaccgtgctgcaccaggactggctgaacggcaaggagtacaagtgcaaggtgagcaacaaggccctgcccgcccccatcgagaagaccatcagcaaggccaagggccagcccagggagccccaggtgtacaccctgccccccagcagggacgagctgaccaagaaccaggtgagcctgacctgcctggtgaagggcttctaccccagcgacatcgccgtggagtgggagagcaacggccagcccgagaacaactacaagaccaccccccccgtgctggacagcgacggcagcttcttcctgtacagcaagctgaccgtggacaagagcaggtggcagcagggcaacgtgttcagctgcagcgtgatgcacgaggccctgcacaaccactacacccagtggagcctgagcctgagccccggcaag

SEQ ID NO: 146 - DNA, 696 bp, synthetic construct
  source 1..696: mol_type = other DNA
gagcccaagagctgcgacaagacccacacctgccccccctgccccgcccccgagctgctgggcggccccagcgtgttcctgttcccccccaagcccaaggacaccctgatgatcagcaggacccccgaggtgacctgcgtggtggtggacgtgagccacgaggaccccgaggtgaagttcaactggtacgtggacggcgtggaggtgcacaacgccaagaccaagcccagggaggagcagtacaacagcacctacagggtggtgagcgtgctgaccgtgctgcaccaggactggctgaacggcaaggagtacaagtgcaaggtgagcaacaaggccctgcccgcccccatcgagaagaccatcagcaaggccaagggccagcccagggagccccaggtgtacaccctgccccccagcagggacgagctgaccaagaaccaggtgagcctgacctgcctggtgtggggcttctaccccagcgacatcgccgtggagtgggagagcaacggccagcccgagaacaactacaagaccaccccccccgtgctggacagcgacggcagcttcttcctgtacagcaagctgaccgtggacaagagcaggtggcagcagggcaacgtgttcagctgcagcgtgatgcacgaggccctgcacaaccactacacccagaagagcctgagcctgagccccggcaag

SEQ ID NO: 147 - DNA, 696 bp, synthetic construct
  source 1..696: mol_type = other DNA
gagcccaagagctgcgacaagacccacacctgccccccctgccccgcccccgagctgctgggcggccccagcgtgttcctgttcccccccaagcccaaggacaccctgatgatcagcaggacccccgaggtgacctgcgtggtggtggacgtgagccacgaggaccccgaggtgaagttcaactggtacgtggacggcgtggaggtgcacaacgccaagaccaagcccagggaggagcagtacaacagcacctacagggtggtgagcgtgctgaccgtgctgcaccaggactggctgaacggcaaggagtacaagtgcaaggtgagcaacaaggccctgcccgcccccatcgagaagaccatcagcaaggccaagggccagcccagggagccccaggtgtacaccctgccccccagcagggacgagctgaccaagaaccaggtgagcctgacctgcctggtgaagggcttctaccccagcgacatcgccgtggagtgggagagcaacggccagcccgagaacaactacaagaccagcccccccgccctggacagcgacggcagcttcgccctggtgagcaagctgaccgtggacaagagcaggtggcagcagggcaacgtgttcagctgcagcgtgatgcacgaggccctgcacaaccactacacccagaagagcctgagcctgagccccggcaag

SEQ ID NO: 148 - DNA, 696 bp, synthetic construct
  source 1..696: mol_type = other DNA
gagcccaagagctgcgacaagacccacacctgccccccctgccccgcccccgagctgctgggcggccccagcgtgttcctgttcccccccaagcccaaggacaccctgatgatcagcaggacccccgaggtgacctgcgtggtggtggacgtgagccacgaggaccccgaggtgaagttcaactggtacgtggacggcgtggaggtgcacaacgccaagaccaagcccagggaggagcagtacaacagcacctacagggtggtgagcgtgctgaccgtgctgcaccaggactggctgaacggcaaggagtacaagtgcaaggtgagcaacaaggccctgcccgcccccatcgagaagaccatcagcaaggccaagggccagcccagggagccccaggtgtacaccctgccccccagcagggacgagctgacctggaaccaggtgagcctgacctgcctggtgaagggcttctaccccagcgacatcgccgtggagtgggagagcaacggccagcccgagaacaactacaagaccaccccccccgtgctggacagcgacggcagcttcttcctgtacagcaagctgaccgtggacaagagcaggtggcagcagggcaacgtgttcagctgcagcgtgatgcacgaggccctgcacaaccactacacccagaagagcctgagcctgagccccggcaag

SEQ ID NO: 149 - protein, 123 aa, synthetic construct
QVQLVESGGGSVQAGGSLRLSCAASGYTYSSTCIGWFRQAPGKDREGVAFAYTGGGVTYADSVKGRFTISQDNAKNTVHLIMNSLKPEDTAMYYCAAKTRGGCWAAAAFYNYWGQGTQVTVSS

SEQ ID NO: 150 - protein, 115 aa, synthetic construct
QVQLVESGGGSVQAGGSLKLSCAASRFIFSRCGMGWFRQAPGKERELVSTISGDGTTFYADSVKGRFTISQHNAATTLYLQMNSLKLEDTAVYYCAADCYNRKYWGQGTQVTVSS

SEQ ID NO: 151 - DNA, 369 bp, synthetic construct
  source 1..369: mol_type = other DNA
caggtgcagctggtggagagcggcggcggcagcgtgcaggccggcggcagcctgaggctgagctgcgccgccagcggctacacctacagcagcacctgcatcggctggttcaggcaggcccccggcaaggacagggagggcgtggccttcgcctacaccggcggcggcgtgacctacgccgacagcgtgaagggcaggttcaccatcagccaggacaacgccaagaacaccgtgcacctgatcatgaacagcctgaagcccgaggacaccgccatgtactactgcgccgccaagaccaggggcggctgctgggccgccgccgccttctacaactactggggccagggcacccaggtgaccgtgagcagc

SEQ ID NO: 152 - DNA, 345 bp, synthetic construct
  source 1..345: mol_type = other DNA
caggtgcagctggtggagagcggcggcggcagcgtgcaggccggcggcagcctgaagctgagctgcgccgccagcaggttcatcttcagcaggtgcggcatgggctggttcaggcaggcccccggcaaggagagggagctggtgagcaccatcagcggcgacggcaccaccttctacgccgacagcgtgaagggcaggttcaccatcagccagcacaacgccgccaccaccctgtacctgcagatgaacagcctgaagctggaggacaccgccgtgtactactgcgccgccgactgctacaacaggaagtactggggccagggcacccaggtgaccgtgagcagc